European Patent Application EP 4 772 193 A1, published July 8, 2026. Title: PHARMACEUTICAL AND ANTI-GPNMB ANTIBODY FOR REMOVING DISEASE-RELATED CELLS. Applicant: TEIJIN PHARMA LIMITED. Application JP. The sequence listing filed with the application follows.

SEQUENCE LISTING (368 sequences)

SEQ ID NO: 1 - protein, 8 aa, Mus musculus
GYAFSNHL

SEQ ID NO: 2 - DNA, 24 bp, synthetic construct
  source 1..24: mol_type = other DNA
ggctacgccttcagcaaccacctg

SEQ ID NO: 3 - protein, 8 aa, Mus musculus
INPGSGGT

SEQ ID NO: 4 - DNA, 24 bp, synthetic construct
  source 1..24: mol_type = other DNA
atcaaccctggcagcggcggcacc

SEQ ID NO: 5 - protein, 12 aa, Mus musculus
ARGANWDVGFAY

SEQ ID NO: 6 - DNA, 36 bp, synthetic construct
  source 1..36: mol_type = other DNA
gctagaggcgctaattgggacgtggggttcgcgtat

SEQ ID NO: 7 - protein, 6 aa, Mus musculus
QDIVKN

SEQ ID NO: 8 - DNA, 18 bp, synthetic construct
  source 1..18: mol_type = other DNA
caagacatcgtgaagaac

SEQ ID NO: 9-10 - skipped (2 entries)

SEQ ID NO: 11 - protein, 9 aa, Mus musculus
LQFHEFPRT

SEQ ID NO: 12 - DNA, 27 bp, synthetic construct
  source 1..27: mol_type = other DNA
ctgcagttccacgagttccctagaacc

SEQ ID NO: 13 - protein, 119 aa, Mus musculus
QVQLQQSGAELVRPGTSVKVSCKASGYAFSNHLIEWVKQRPGQGLEWIGVINPGSGGTNYIEKFKGKATLTADKSSSTAYMQLSSLTSDDSAVYFCARGANWDVGFAYWGQGTLVTVSA

SEQ ID NO: 14 - DNA, 357 bp, synthetic construct
  source 1..357: mol_type = other DNA
caagtgcagctgcagcaatctggcgccgagctggtgagacctggcacaagcgtgaaggtgagctgcaaggctagcggctacgccttcagcaaccacctgatcgagtgggtgaagcagagacctggccaaggcctggagtggatcggcgtgatcaaccctggcagcggcggcaccaactacatcgagaagttcaagggcaaggccaccctgaccgccgacaagagcagcagcaccgcctacatgcagctgagcagcctgacaagcgacgacagcgccgtgtacttctgcgctagaggcgctaattgggacgtggggttcgcgtattggggccaaggcaccctggtgaccgtgagcgcc

SEQ ID NO: 15 - protein, 107 aa, Mus musculus
EIQMTQSPSSMSASLGDRITITCQATQDIVKNLNWYQQKPGKPPSFLIYYATELAEGVPSRFSGSGSGSDFSLTISNLESEDFADYYCLQFHEFPRTFGGGTKLEIK

SEQ ID NO: 16 - DNA, 321 bp, synthetic construct
  source 1..321: mol_type = other DNA
gagattcagatgacacagagccctagcagcatgagcgctagcctgggcgacagaatcaccatcacctgccaagccacccaagacatcgtgaagaacctgaactggtatcagcagaagcctggcaagcctcctagcttcctgatctactacgccaccgagctggccgagggcgtgcctagcagattcagcggcagcggcagcggcagcgacttcagcctgaccatcagcaacctggagagcgaggacttcgccgactactactgcctgcagttccacgagttccctagaaccttcggcggcggcaccaagctggagatcaag

SEQ ID NO: 17 - protein, 8 aa, Mus musculus
GYTFTDNW

SEQ ID NO: 18 - DNA, 24 bp, synthetic construct
  source 1..24: mol_type = other DNA
ggctacaccttcaccgacaactgg

SEQ ID NO: 19 - protein, 8 aa, Mus musculus
IDPSDSFT

SEQ ID NO: 20 - DNA, 24 bp, synthetic construct
  source 1..24: mol_type = other DNA
atcgaccctagcgacagcttcacc

SEQ ID NO: 21 - protein, 15 aa, Mus musculus
TRSGYYGSPKLGGDY

SEQ ID NO: 22 - DNA, 45 bp, synthetic construct
  source 1..45: mol_type = other DNA
acaagaagcggctactatggctcccctaaattgggcggcgactac

SEQ ID NO: 23 - protein, 5 aa, Mus musculus
SSISY

SEQ ID NO: 24 - DNA, 15 bp, synthetic construct
  source 1..15: mol_type = other DNA
agcagcatcagctac

SEQ ID NO: 25-26 - skipped (2 entries)

SEQ ID NO: 27 - protein, 9 aa, Mus musculus
HQWNSYPCT

SEQ ID NO: 28 - DNA, 27 bp, synthetic construct
  source 1..27: mol_type = other DNA
catcagtggaacagctacccttgcacc

SEQ ID NO: 29 - protein, 122 aa, Mus musculus
QVQLQQPGAEIVRPGASVKLSCKASGYTFTDNWMGWVKQRPGQGLEWIGAIDPSDSFTNYNQNFKGKATLTVDTSSSTAYMQLSSLTSEDSAVYFCTRSGYYGSPKLGGDYWGQGTTLTVSS

SEQ ID NO: 30 - DNA, 366 bp, synthetic construct
  source 1..366: mol_type = other DNA
caagtgcagctgcagcagcctggcgccgagatcgtgagacctggcgctagcgtgaagctgagctgcaaggctagcggctacaccttcaccgacaactggatgggctgggtgaagcagagacctggccaaggcctggagtggatcggcgccatcgaccctagcgacagcttcaccaactacaatcagaacttcaagggcaaggcgacgttaaccgtcgacacaagcagcagcaccgcctacatgcagctgagcagcctgacaagcgaggacagcgccgtgtacttctgcacaagaagcggctactatggctcccctaaattgggcggcgactactggggccaaggcaccacactgacggttagctcc

SEQ ID NO: 31 - protein, 106 aa, Mus musculus
QIVLTQSPAIMSASLGEEITLTCSASSSISYMHWYQQKSGTSPKLLIYSTSNLASGVPSRFSGSGSGTFYSLTISSVEAEDAADYYCHQWNSYPCTFGGGTKLEIK

SEQ ID NO: 32 - DNA, 318 bp, synthetic construct
  source 1..318: mol_type = other DNA
cagatcgtgctgacacagagccctgccatcatgagcgctagcctgggcgaggagatcaccctgacctgcagcgctagcagcagcatcagctacatgcactggtatcagcagaagagcggtacaagccctaagctgctgatctacagcacaagcaacctggctagcggcgtgcctagcagattcagcggcagcggcagcggcaccttctacagcctgaccatcagcagcgtggaggccgaggacgccgccgactactactgccatcagtggaacagctacccttgcaccttcggcggcggcaccaagctggagatcaag

SEQ ID NO: 33 - protein, 8 aa, Mus musculus
GYTFTDYW

SEQ ID NO: 34 - DNA, 24 bp, synthetic construct
  source 1..24: mol_type = other DNA
ggctacaccttcaccgactactgg

SEQ ID NO: 35 - protein, 8 aa, Mus musculus
IDPSDSYT

SEQ ID NO: 36 - DNA, 24 bp, synthetic construct
  source 1..24: mol_type = other DNA
atcgaccctagcgacagctacacc

SEQ ID NO: 37 - protein, 15 aa, Mus musculus
ARSGYYGSPKLGGDY

SEQ ID NO: 38 - DNA, 45 bp, synthetic construct
  source 1..45: mol_type = other DNA
gctagaagcggctactatggctcccctaaattgggcggcgactac

SEQ ID NO: 39 - protein, 5 aa, Mus musculus
SSISY

SEQ ID NO: 40 - DNA, 15 bp, synthetic construct
  source 1..15: mol_type = other DNA
agcagcatcagctac

SEQ ID NO: 41-42 - skipped (2 entries)

SEQ ID NO: 43 - protein, 9 aa, Mus musculus
HQWNSYPCT

SEQ ID NO: 44 - DNA, 27 bp, synthetic construct
  source 1..27: mol_type = other DNA
catcagtggaacagctacccttgcacc

SEQ ID NO: 45 - protein, 122 aa, Mus musculus
QVQLQQPGAEIVRPGASVKLSCKASGYTFTDYWMNWVKQRPGQGLEWIGAIDPSDSYTNYNQEFNGKATLTVDTSSSTAYMQLSSLTSEDSAVYFCARSGYYGSPKLGGDYWGQGTTLTVSS

SEQ ID NO: 46 - DNA, 366 bp, synthetic construct
  source 1..366: mol_type = other DNA
caagtgcagctgcagcagcctggcgccgagatcgtgagacctggcgctagcgtgaagctgagctgcaaggctagcggctacaccttcaccgactactggatgaactgggtgaagcagagacctggccaaggcctggagtggatcggcgccatcgaccctagcgacagctacaccaactacaaccaagagttcaacggcaaggcgacgttaaccgtcgacacaagcagcagcaccgcctacatgcagctgagcagcctgacaagcgaggacagcgccgtgtacttctgcgctagaagcggctactatggctcccctaaattgggcggcgactactggggccaaggcaccacactgacggttagctcc

SEQ ID NO: 47 - protein, 106 aa, Mus musculus; identical to SEQ ID NO: 31

SEQ ID NO: 48 - DNA, 318 bp, synthetic construct; identical to SEQ ID NO: 32
  source 1..318: mol_type = other DNA

SEQ ID NO: 49 - protein, 8 aa, Mus musculus
GYTFTDCY

SEQ ID NO: 50 - DNA, 24 bp, synthetic construct
  source 1..24: mol_type = other DNA
gggtacacctttaccgactgctac

SEQ ID NO: 51 - protein, 8 aa, Mus musculus
INPNSGYT

SEQ ID NO: 52 - DNA, 24 bp, synthetic construct
  source 1..24: mol_type = other DNA
atcaaccccaacagtggctacacg

SEQ ID NO: 53 - protein, 16 aa, Mus musculus
TRGDYYTSNLYDWFAY

SEQ ID NO: 54 - DNA, 48 bp, synthetic construct
  source 1..48: mol_type = other DNA
acaagaggcgattactacacctccaatctctatgactggtttgcatac

SEQ ID NO: 55 - protein, 6 aa, Mus musculus
QTVGTV

SEQ ID NO: 56 - DNA, 18 bp, synthetic construct
  source 1..18: mol_type = other DNA
cagaccgtagggactgtg

SEQ ID NO: 57-58 - skipped (2 entries)

SEQ ID NO: 59 - protein, 9 aa, Mus musculus
LQYGSVPPT

SEQ ID NO: 60 - DNA, 27 bp, synthetic construct
  source 1..27: mol_type = other DNA
ctgcagtatggcagcgttccacccacc

SEQ ID NO: 61 - protein, 123 aa, Mus musculus
QVNLLQSGAALVKPGASVRLSCKTSGYTFTDCYIHWVRQSHGKSLEWIGFINPNSGYTFYNEKFKSKATLTVAKSTNTAYMELSRLTSEDSATYFCTRGDYYTSNLYDWFAYWGQGTLVTVSS

SEQ ID NO: 62 - DNA, 369 bp, synthetic construct
  source 1..369: mol_type = other DNA
caggtcaatctgctgcagtccggagctgcattggtcaaacccggagccagcgtacggctttcctgtaagacatctgggtacacctttaccgactgctacattcactgggtaaggcagtcacatgggaagagccttgagtggattggcttcatcaaccccaacagtggctacacgttctacaacgagaagttcaagtccaaagctacactgacagtggccaaaagcaccaacactgcctatatggagctgtcacgcttgacatccgaagatagtgccacatatttctgcacaagaggcgattactacacctccaatctctatgactggtttgcatactggggtcaaggcaccctggttaccgtgtcatct

SEQ ID NO: 63 - protein, 107 aa, Mus musculus
DTVMTQSPASMSTSVGERVTVNCKASQTVGTVVAWFQQKPGQSPKRLIYWATNRHTGVPDRFTGSGFGRDFSLTISNVEAEDLAVYYCLQYGSVPPTFGGGTKLELK

SEQ ID NO: 64 - DNA, 321 bp, synthetic construct
  source 1..321: mol_type = other DNA
gacacagtcatgacccaatcaccagcatccatgagcacttcagttggcgagagagtgaccgtgaactgtaaggcctctcagaccgtagggactgtggttgcctggttccagcagaaaccagggcaaagccccaaacggctgatatactgggcaacgaatcgacacactggtgtacctgaccgctttaccggcagtgggttcggaagggacttctccctcaccatttccaacgtcgaagccgaagatcttgccgtgtactattgcctgcagtatggcagcgttccacccacctttggaggaggcacaaagttggagctgaag

SEQ ID NO: 65 - protein, 8 aa, Mus musculus
GYTFTNHN

SEQ ID NO: 66 - DNA, 24 bp, synthetic construct
  source 1..24: mol_type = other DNA
ggctacacatttaccaatcacaat

SEQ ID NO: 67 - protein, 8 aa, Mus musculus
FYTGNGDT

SEQ ID NO: 68 - DNA, 24 bp, synthetic construct
  source 1..24: mol_type = other DNA
ttttatacaggaaatggtgatact

SEQ ID NO: 69 - protein, 14 aa, Mus musculus
ARERYDGYYIAMDY

SEQ ID NO: 70 - DNA, 42 bp, synthetic construct
  source 1..42: mol_type = other DNA
gcaagagaaaggtatgatggttactatattgctatggactac

SEQ ID NO: 71 - protein, 5 aa, Mus musculus
SSVYY

SEQ ID NO: 72 - DNA, 15 bp, synthetic construct
  source 1..15: mol_type = other DNA
tcgagtgtgtattac

SEQ ID NO: 73-74 - skipped (2 entries)

SEQ ID NO: 75 - protein, 10 aa, Mus musculus
QQWSSNPQWT

SEQ ID NO: 76 - DNA, 30 bp, synthetic construct
  source 1..30: mol_type = other DNA
cagcagtggagtagtaacccacagtggacg

SEQ ID NO: 77 - protein, 121 aa, Mus musculus
QVQLQQPGAELVKPGASVKMSCKASGYTFTNHNMHWVKQTPGQGLEWIGAFYTGNGDTSYNQKFKGKATLTADKSSSTAYIQLSSLTSEDSAVYYCARERYDGYYIAMDYWGQGTSVTVSS

SEQ ID NO: 78 - DNA, 363 bp, synthetic construct
  source 1..363: mol_type = other DNA
caggtacaactgcagcagcctggggctgagctggtgaagcctggggcctcagtgaagatgtcctgcaaggcttctggctacacatttaccaatcacaatatgcactgggtaaagcagacacctggacagggcctggaatggattggagctttttatacaggaaatggtgatacttcctacaatcagaagttcaagggcaaggccacattgactgcagacaaatcctccagcacagcctacatacaactcagcagcctgacatctgaggactctgcggtctattactgtgcaagagaaaggtatgatggttactatattgctatggactactggggtcaaggaacctcagtcaccgtctcctca

SEQ ID NO: 79 - protein, 107 aa, Mus musculus
QIVLTQSPAFMSVSPGEKVTMTCSASSSVYYMFWYQQKPRSSPKPWIYLTSKLASGVPARFSGSGSGTSYSVTISSMEAEDAATYYCQQWSSNPQWTFGGGTKLEIK

SEQ ID NO: 80 - DNA, 321 bp, synthetic construct
  source 1..321: mol_type = other DNA
caaattgttctcacccagtctccagcattcatgtctgtatctccaggggagaaggtcaccatgacctgcagtgccagctcgagtgtgtattacatgttctggtaccagcagaagccaagatcctcccccaaaccctggatttatctcacatccaagctggcttctggagtccctgctcgcttcagtggcagtgggtctgggacctcttactctgtcacaatcagcagcatggaggctgaagatgctgccacttattactgccagcagtggagtagtaacccacagtggacgttcggtggaggcaccaagctggaaatcaaa

SEQ ID NO: 81 - protein, 10 aa, Mus musculus
GFSLTTSGMG

SEQ ID NO: 82 - DNA, 30 bp, synthetic construct
  source 1..30: mol_type = other DNA
gggttttcactgaccacttctggtatgggt

SEQ ID NO: 83 - protein, 7 aa, Mus musculus
MWWDDDK

SEQ ID NO: 84 - DNA, 21 bp, synthetic construct
  source 1..21: mol_type = other DNA
atgtggtgggatgacgataag

SEQ ID NO: 85 - protein, 11 aa, Mus musculus
ARRVYSSWFAY

SEQ ID NO: 86 - DNA, 33 bp, synthetic construct
  source 1..33: mol_type = other DNA
gctcgaagagtctacagtagttggtttgcttac

SEQ ID NO: 87 - protein, 6 aa, Mus musculus
QNVGAN

SEQ ID NO: 88 - DNA, 18 bp, synthetic construct
  source 1..18: mol_type = other DNA
cagaatgtgggtgctaat

SEQ ID NO: 89-90 - skipped (2 entries)

SEQ ID NO: 91 - protein, 9 aa, Mus musculus
QQYNNYPLT

SEQ ID NO: 92 - DNA, 27 bp, synthetic construct
  source 1..27: mol_type = other DNA
cagcaatataacaactatcctctcacg

SEQ ID NO: 93 - protein, 119 aa, Mus musculus
QVTLKESGPGILQPSQTLSLTCSFSGFSLTTSGMGVGWIRQPSGKGLEWLADMWWDDDKNYNPSLKSRLTISKDNSKKQVFLKIASVDTADTATYYCARRVYSSWFAYWGQGTLVTVSA

SEQ ID NO: 94 - DNA, 357 bp, synthetic construct
  source 1..357: mol_type = other DNA
caggttactctgaaagagtctggccctggaatattgcagccctcccagaccctcagtctgacttgttctttctctgggttttcactgaccacttctggtatgggtgtaggctggattcgtcagccttcaggaaagggtctagagtggctggcagacatgtggtgggatgacgataagaattataatccatccctgaagagccggctcacaatctccaaggataactccaaaaagcaggtattcctcaagatcgccagtgtggacactgcagatactgccacttactactgtgctcgaagagtctacagtagttggtttgcttactggggccaagggactctggtcactgtctctgca

SEQ ID NO: 95 - protein, 109 aa, Mus musculus
DGDIVMTQSQKFMSTSVGDRVSVTCKASQNVGANVAWYQQKPGQSPKTLIYSASYRYGGVPDRFTGSGSGTDFTFTITNVQSEDLAEYFCQQYNNYPLTFGAGTKLDLK

SEQ ID NO: 96 - DNA, 327 bp, synthetic construct
  source 1..327: mol_type = other DNA
gatggagacattgtgatgacccagtctcaaaaattcatgtccacatcagtaggagacagggtcagcgtcacctgcaaggccagtcagaatgtgggtgctaatgtagcctggtatcaacagaaaccagggcaatctcctaaaacactgatttattcggcatcctaccggtacggtggagtccctgatcgcttcacaggcagtggatctgggacagatttcactttcaccatcactaatgtgcagtctgaagacttggcagagtatttctgtcagcaatataacaactatcctctcacgttcggtgctgggaccaagttggacctgaaa

SEQ ID NO: 97 - protein, 8 aa, Mus musculus
GYTLSSYW

SEQ ID NO: 98 - DNA, 24 bp, synthetic construct
  source 1..24: mol_type = other DNA
ggctacactttaagtagttattgg

SEQ ID NO: 99 - protein, 8 aa, Mus musculus
INPSNNYT

SEQ ID NO: 100 - DNA, 24 bp, synthetic construct
  source 1..24: mol_type = other DNA
attaatcctagcaataattatact

SEQ ID NO: 101 - protein, 5 aa, Mus musculus
ATWGY

SEQ ID NO: 102 - DNA, 15 bp, synthetic construct
  source 1..15: mol_type = other DNA
gcaacatggggctac

SEQ ID NO: 103 - protein, 6 aa, Mus musculus
QDVSTA

SEQ ID NO: 104 - DNA, 18 bp, synthetic construct
  source 1..18: mol_type = other DNA
caggatgtgagtactgct

SEQ ID NO: 105-106 - skipped (2 entries)

SEQ ID NO: 107 - protein, 9 aa, Mus musculus
QHHYTTTWT

SEQ ID NO: 108 - DNA, 27 bp, synthetic construct
  source 1..27: mol_type = other DNA
cagcaccattatactactacgtggacg

SEQ ID NO: 109 - protein, 112 aa, Mus musculus
QVQLQQSGAELTKPGTSVKMSCKASGYTLSSYWMNWIKQRPGQGLEWIGTINPSNNYTAYNLKFKDKAMLTADKSSSTAYMQLSSLTSEDSAVYYCATWGYWGQGTTLTVSS

SEQ ID NO: 110 - DNA, 336 bp, synthetic construct
  source 1..336: mol_type = other DNA
caggtccagctgcagcagtctggcgctgaactgacaaaacctgggacctcagtgaagatgtcctgcaaggcctctggctacactttaagtagttattggatgaactggataaaacagaggcctggacaaggtctggaatggattgggactattaatcctagcaataattatactgcatacaatctgaagtttaaggacaaggccatgttgactgcagacaaatcctccagtacagcctacatgcaactcagcagcctgacatctgaggactctgcagtctattactgtgcaacatggggctactggggccaaggcaccactctcacagtctcctca

SEQ ID NO: 111 - protein, 107 aa, Mus musculus
DIVMTQSHKFMSTSVGDRVSITCKASQDVSTAVAWHQQKPGQPPKLLIYSASYRYTGVPDRFTGSGSGTDFTFTISSVQTEDLAIYYCQHHYTTTWTFGGGTKLEIR

SEQ ID NO: 112 - DNA, 321 bp, synthetic construct
  source 1..321: mol_type = other DNA
gacattgtgatgacccagtctcacaaattcatgtccacatcagtaggagacagggtcagcatcacctgcaaggccagtcaggatgtgagtactgctgtagcctggcatcaacagaaaccaggacagcctcctaagctactgatttactcggcatcttaccggtacactggagtccctgatcgcttcactggcagtggatctgggacggatttcactttcaccatcagcagtgtgcagactgaagacctggcaatttattactgtcagcaccattatactactacgtggacgttcggtggaggcaccaagctggaaatcaga

SEQ ID NO: 113 - protein, 10 aa, Mus musculus
GFSLSTSVMG

SEQ ID NO: 114 - DNA, 30 bp, synthetic construct
  source 1..30: mol_type = other DNA
ggcttctctctgtccacatctgtgatgggc

SEQ ID NO: 115 - protein, 7 aa, Mus musculus
IWWDDDK

SEQ ID NO: 116 - DNA, 21 bp, synthetic construct
  source 1..21: mol_type = other DNA
atctggtgggacgacgataag

SEQ ID NO: 117 - protein, 15 aa, Mus musculus
ARAYYSNYEYYGMDY

SEQ ID NO: 118 - DNA, 45 bp, synthetic construct
  source 1..45: mol_type = other DNA
gcccgcgcttattactctaactacgagtactatggcatggattac

SEQ ID NO: 119 - protein, 11 aa, Mus musculus
QSIVHSNGNTY

SEQ ID NO: 120 - DNA, 33 bp, synthetic construct
  source 1..33: mol_type = other DNA
cagagcattgttcatagtaatggaaacacctat

SEQ ID NO: 121-122 - skipped (2 entries)

SEQ ID NO: 123 - protein, 9 aa, Mus musculus
FQGSHVPFT

SEQ ID NO: 124 - DNA, 27 bp, synthetic construct
  source 1..27: mol_type = other DNA
tttcaaggttcacatgttccattcacg

SEQ ID NO: 125 - protein, 123 aa, Mus musculus
QVTLKESGPGILQPSQTLSLTCSFSGFSLSTSVMGVGWIRQPSGKGLEWLADIWWDDDKDYNPSLKSRLTISKDTSKNQVFLKIASVDTADTATYYCARAYYSNYEYYGMDYWGQGTSVTVSS

SEQ ID NO: 126 - DNA, 369 bp, synthetic construct
  source 1..369: mol_type = other DNA
caggtcacactgaaagagtctggtcccggcatcctgcagccttctcagaccctgtctctgacctgtagcttctccggcttctctctgtccacatctgtgatgggcgtgggctggatcagacagccttctggcaagggcctggagtggctggctgacatctggtgggacgacgataaggattacaacccttccctgaagtctcggctgaccatcagcaaggatacatccaagaatcaggtgttcctgaagatcgcttctgtggacaccgccgacaccgccacatattactgtgcccgcgcttattactctaactacgagtactatggcatggattactggggccagggcacatctgtgacagtgtcttcc

SEQ ID NO: 127 - protein, 112 aa, Mus musculus
DVLMTQTPLSLPVSLGDQASISCRSSQSIVHSNGNTYLEWYLQKPGQSPKLLIYKVSNRFSGVPDRFSGSGSGTDFTLKISRVEAEDLGVYYCFQGSHVPFTFGSGTKLEIK

SEQ ID NO: 128 - DNA, 336 bp, synthetic construct
  source 1..336: mol_type = other DNA
gatgttttgatgacccaaactccactctccctgcctgtcagtcttggagatcaagcctccatctcttgcagatctagtcagagcattgttcatagtaatggaaacacctatttagaatggtacctgcagaaaccaggccagtctccaaagctcctgatctacaaggtttccaaccgattttctggggtcccagacaggttcagtggcagtggatcagggacagatttcacactcaagatcagcagagtggaggctgaggatctgggagtttattactgctttcaaggttcacatgttccattcacgttcggctcggggacaaagttggaaataaaa

SEQ ID NO: 129 - protein, 10 aa, Mus musculus
GFSLSTSVMG

SEQ ID NO: 130 - DNA, 24 bp, synthetic construct
  source 1..24: mol_type = other DNA
gggttttcactgagtacttctgtt

SEQ ID NO: 131 - protein, 7 aa, Mus musculus
IWWDDDK

SEQ ID NO: 132 - DNA, 21 bp, synthetic construct
  source 1..21: mol_type = other DNA
atttggtgggatgacgataag

SEQ ID NO: 133 - protein, 15 aa, Mus musculus
ARTYYSNYEYYGMDY

SEQ ID NO: 134 - DNA, 45 bp, synthetic construct
  source 1..45: mol_type = other DNA
gctcgaacctactatagtaactacgaatactatggtatggactac

SEQ ID NO: 135 - protein, 11 aa, Mus musculus
QTIILSNGNTY

SEQ ID NO: 136 - DNA, 33 bp, synthetic construct
  source 1..33: mol_type = other DNA
cagaccattatacttagtaatggaaacacctat

SEQ ID NO: 137-138 - skipped (2 entries)

SEQ ID NO: 139 - protein, 9 aa, Mus musculus
FQGSHVPFT

SEQ ID NO: 140 - DNA, 27 bp, synthetic construct
  source 1..27: mol_type = other DNA
tttcaaggttcacatgttccattcacg

SEQ ID NO: 141 - protein, 123 aa, Mus musculus
QVTLKESGPGILQPSQTLSLTCSFSGFSLSTSVMGVGWIRQPSGKGLEWLADIWWDDDKDYNPSLKSRLTISKDTSKNQVFLKIASVDTADTATYYCARTYYSNYEYYGMDYWGQGTSVTVSS

SEQ ID NO: 142 - DNA, 369 bp, synthetic construct
  source 1..369: mol_type = other DNA
caggttactctgaaagagtctggccctggaatattgcagccctcccagaccctcagtctgacttgttctttctctgggttttcactgagtacttctgttatgggtgtaggctggattcgtcagccttcaggaaagggtctagagtggctggcagacatttggtgggatgacgataaggactataacccatccctgaagagccggctcacaatctccaaggatacctccaaaaaccaggtattcctcaagatcgccagtgtggacactgcagatactgccacttactactgtgctcgaacctactatagtaactacgaatactatggtatggactactggggtcaaggaacctcagtcaccgtctcctca

SEQ ID NO: 143 - protein, 112 aa, Mus musculus
DVLMTQTPLSLPVSLGDQASISCRSSQTIILSNGNTYLEWYLQKPGQSPKLLIYKVSNRFSGVPDRFSGSGSGTDFTLKISRVEAEDLGVYYCFQGSHVPFTFGSGTKLEIK

SEQ ID NO: 144 - DNA, 336 bp, synthetic construct
  source 1..336: mol_type = other DNA
gacgttttgatgacccaaactccactctccctgcctgtcagtcttggagatcaagcctccatctcttgcagatctagtcagaccattatacttagtaatggaaacacctatttagaatggtacctgcagaaaccaggccagtctccaaagctcctgatctacaaagtttccaaccgattttctggggtcccagacaggttcagtggcagtggatcggggacagatttcacactcaagatcagcagagtggaggctgaggatctgggagtttattactgttttcaaggttcacatgttccattcacgttcggctcggggacaaagttagaaataaaa

SEQ ID NO: 145 - protein, 8 aa, Mus musculus
GYTFTDYY

SEQ ID NO: 146 - DNA, 24 bp, synthetic construct
  source 1..24: mol_type = other DNA
ggatacacattcactgactactac

SEQ ID NO: 147 - protein, 8 aa, Mus musculus
INPINGDI

SEQ ID NO: 148 - DNA, 24 bp, synthetic construct
  source 1..24: mol_type = other DNA
attaatccgatcaatggtgatatt

SEQ ID NO: 149 - protein, 15 aa, Mus musculus
AREAFFGYKGNYFDY

SEQ ID NO: 150 - DNA, 45 bp, synthetic construct
  source 1..45: mol_type = other DNA
gcaagagaggctttctttggttacaaggggaactactttgactac

SEQ ID NO: 151 - protein, 10 aa, Mus musculus
ESVDNYGISF

SEQ ID NO: 152 - DNA, 30 bp, synthetic construct
  source 1..30: mol_type = other DNA
gaaagtgttgataattatggcattagtttt

SEQ ID NO: 153-154 - skipped (2 entries)

SEQ ID NO: 155 - protein, 9 aa, Mus musculus
QQTKEVPYT

SEQ ID NO: 156 - DNA, 27 bp, synthetic construct
  source 1..27: mol_type = other DNA
cagcaaactaaggaggttccgtacacg

SEQ ID NO: 157 - protein, 122 aa, Mus musculus
EVQLQQSGPELVMPGSSVKISCKASGYTFTDYYMNWVRQSHGKSLEWIGDINPINGDITYNQKFKGKATLTVDKSSSTDYMELRGLTSEDSAVYYCAREAFFGYKGNYFDYWGQGTTLTVSS

SEQ ID NO: 158 - DNA, 366 bp, synthetic construct
  source 1..366: mol_type = other DNA
gaggtccagctgcaacagtctgggcctgagctggtgatgcctgggtcttcagtgaagatatcatgtaaggcttctggatacacattcactgactactacatgaactgggtgaggcagagccatggaaagagccttgagtggattggagatattaatccgatcaatggtgatattacctacaaccagaagttcaagggcaaggccacattgactgtagacaagtcctccagcacagactacatggagctccgcggcctgacatctgaggactctgcagtctattactgtgcaagagaggctttctttggttacaaggggaactactttgactactggggccaaggcaccactctcacagtctcctca

SEQ ID NO: 159 - protein, 111 aa, Mus musculus
DIVLTQSPASLAVSLGQRATISCRASESVDNYGISFMSWFQQKPGQPPKLLIYAASNQGSGVPAKFSGSGSGTDFSLNIHPMEEDDPAMYFCQQTKEVPYTFGGGTKLEIK

SEQ ID NO: 160 - DNA, 333 bp, synthetic construct
  source 1..333: mol_type = other DNA
gacattgtgctgacccaatctccagcttctttggctgtgtctctagggcagagggccaccatctcctgcagagccagcgaaagtgttgataattatggcattagttttatgagctggttccaacagaaaccaggacagccacccaaactcctcatctatgctgcatccaaccaaggatccggggtccctgccaagtttagtggcagtgggtctgggacagacttcagcctcaacatccatcctatggaggaggatgatcctgcaatgtatttctgtcagcaaactaaggaggttccgtacacgttcggaggggggaccaagctggaaataaaa

SEQ ID NO: 161 - protein, 10 aa, Mus musculus
GFSLSTSVMG

SEQ ID NO: 162 - DNA, 30 bp, synthetic construct
  source 1..30: mol_type = other DNA
gggttttcactgagtacttctgttatgggt

SEQ ID NO: 163 - protein, 7 aa, Mus musculus
IWWDDDK

SEQ ID NO: 164 - DNA, 21 bp, synthetic construct
  source 1..21: mol_type = other DNA
atttggtgggatgacgataag

SEQ ID NO: 165 - protein, 15 aa, Mus musculus
ARAYYSNFEYYGMDY

SEQ ID NO: 166 - DNA, 45 bp, synthetic construct
  source 1..45: mol_type = other DNA
gctcgagcctactatagtaacttcgaatactatggtatggactac

SEQ ID NO: 167 - protein, 11 aa, Mus musculus
QTIVHSNGNTY

SEQ ID NO: 168 - DNA, 33 bp, synthetic construct
  source 1..33: mol_type = other DNA
cagaccattgtacatagtaatggaaacacctat

SEQ ID NO: 169-170 - skipped (2 entries)

SEQ ID NO: 171 - protein, 9 aa, Mus musculus
FQGSHVPFT

SEQ ID NO: 172 - DNA, 27 bp, synthetic construct
  source 1..27: mol_type = other DNA
tttcaaggttcacatgttccattcacg

SEQ ID NO: 173 - protein, 123 aa, Mus musculus
QVTLKESGPGILQPSQTLSLTCSFSGFSLSTSVMGVGWIRQPSGKGLEWLADIWWDDDKDYNPSLKSRLTISKDTSKNQVFLKIASVDTADTATYYCARAYYSNFEYYGMDYWGQGTSVTVSS

SEQ ID NO: 174 - DNA, 369 bp, synthetic construct
  source 1..369: mol_type = other DNA
caggttactctgaaagagtctggccctggaatattgcagccctcccagaccctcagtctgacttgttctttctctgggttttcactgagtacttctgttatgggtgtaggctggattcgtcagccttcaggaaagggtcttgagtggctggcagacatttggtgggatgacgataaggactataacccatctctgaagagccggctcacaatctccaaggatacctccaaaaaccaggtattcctcaagatcgccagtgtggacactgcagatactgccacttactactgtgctcgagcctactatagtaacttcgaatactatggtatggactactggggtcaaggaacctcagtcaccgtctcctca

SEQ ID NO: 175 - protein, 112 aa, Mus musculus
DVLMTQIPLSLPVSLGDQASISCRSSQTIVHSNGNTYLEWYLQKPGQSPKLLIYKVSNRFSGVPDRFSGSGSGTDFTLKISRVEAEDLGVYYCFQGSHVPFTFGSGTKLEIK

SEQ ID NO: 176 - DNA, 336 bp, synthetic construct
  source 1..336: mol_type = other DNA
gatgttttgatgacccaaattccactctccctgcctgtcagtcttggagatcaagcctccatctcttgcagatctagtcagaccattgtacatagtaatggaaacacctatttagaatggtacctgcagaaaccaggccagtctccaaagctcctgatctacaaagtttccaaccgattttctggggtcccagacaggttcagtggcagtggatcggggacagatttcacactcaagatcagcagagtggaggctgaggatctgggagtttattactgctttcaaggttcacatgttccattcacgttcggctcggggacaaagttggaaataaaa

SEQ ID NO: 177 - protein, 10 aa, Mus musculus
GYTFTTYWMN

SEQ ID NO: 178 - DNA, 30 bp, synthetic construct
  source 1..30: mol_type = other DNA
ggctacacctttactacctactggatgaac

SEQ ID NO: 179 - protein, 8 aa, Mus musculus
INPSNDYT

SEQ ID NO: 180 - DNA, 24 bp, synthetic construct
  source 1..24: mol_type = other DNA
attaatcctagcaatgattatact

SEQ ID NO: 181 - protein, 8 aa, Mus musculus
GRSYSPDY

SEQ ID NO: 182 - DNA, 24 bp, synthetic construct
  source 1..24: mol_type = other DNA
ggaaggagttactcccctgactac

SEQ ID NO: 183 - protein, 6 aa, Mus musculus
QNVDNH

SEQ ID NO: 184 - DNA, 18 bp, synthetic construct
  source 1..18: mol_type = other DNA
cagaatgtggataatcat

SEQ ID NO: 185-186 - skipped (2 entries)

SEQ ID NO: 187 - protein, 9 aa, Mus musculus
QQYKSYPFT

SEQ ID NO: 188 - DNA, 27 bp, synthetic construct
  source 1..27: mol_type = other DNA
cagcaatataaaagctatccattcacg

SEQ ID NO: 189 - protein, 115 aa, Mus musculus
QVQLQQSGAELAKPGTSVKMSCKASGYTFTTYWMNWVKQRPGQDLEWIGAINPSNDYTEYNQKFKDKAILTADKSSNTAYMQLSSLTSEDSAVYYCGRSYSPDYWGQGTTLTVSS

SEQ ID NO: 190 - DNA, 345 bp, synthetic construct
  source 1..345: mol_type = other DNA
caggtccagctgcagcagtctggcgctgaactggcaaaacctgggacctcagtgaagatgtcctgcaaggcttctggctacacctttactacctactggatgaactgggtaaaacagaggcctggacaggatctggaatggattggggctattaatcctagcaatgattatactgagtacaatcagaagttcaaggacaaggccatattgactgcagacaaatcctccaacacagcctacatgcaactgagtagcctgacatctgaggactctgcagtctattactgtggaaggagttactcccctgactactggggccaaggcaccactctcacagtctcatca

SEQ ID NO: 191 - protein, 107 aa, Mus musculus
DIVMTQSQKFMSTSVGDRVSVTCKASQNVDNHVAWHQQKPGQSPKALIYSASYRYSGVPDRFTGSGSGTDFTLTIRDVQSEDLADYFCQQYKSYPFTFGSGTELEIK

SEQ ID NO: 192 - DNA, 321 bp, synthetic construct
  source 1..321: mol_type = other DNA
gacattgtgatgacccagtctcaaaaattcatgtccacatcagtaggagacagggtcagcgtcacctgcaaggccagtcagaatgtggataatcatgtagcctggcatcaacagaaaccagggcagtctcctaaggcactgatttactcggcatcctaccggtacagtggagtccctgatcgcttcacaggcagtggatctgggacagatttcactctcaccatccgcgatgtgcagtctgaagacttggcagactatttctgtcagcaatataaaagctatccattcacgttcggctcggggacagagttggaaataaaa

SEQ ID NO: 193 - protein, 8 aa, Mus musculus
GFNIKDYY

SEQ ID NO: 194 - DNA, 24 bp, synthetic construct
  source 1..24: mol_type = other DNA
ggcttcaacattaaagactactat

SEQ ID NO: 195 - protein, 8 aa, Mus musculus
IDPENGDT

SEQ ID NO: 196 - DNA, 24 bp, synthetic construct
  source 1..24: mol_type = other DNA
attgatcctgagaatggtgatact

SEQ ID NO: 197 - protein, 13 aa, Mus musculus
NGVYYGSRGFFDY

SEQ ID NO: 198 - DNA, 39 bp, synthetic construct
  source 1..39: mol_type = other DNA
aatggagtttactacggtagtagagggttctttgactac

SEQ ID NO: 199 - protein, 11 aa, Mus musculus
QSLLDSDGKTY

SEQ ID NO: 200 - DNA, 33 bp, synthetic construct
  source 1..33: mol_type = other DNA
cagagcctcttagatagtgatggaaagacatat

SEQ ID NO: 201-202 - skipped (2 entries)

SEQ ID NO: 203 - protein, 9 aa, Mus musculus
CQITHFPFT

SEQ ID NO: 204 - DNA, 27 bp, synthetic construct
  source 1..27: mol_type = other DNA
tgccaaattacacattttccattcacg

SEQ ID NO: 205 - protein, 120 aa, Mus musculus
EVQLQQSGAELVRSGASVKLSCTASGFNIKDYYMHWVKQRPDQGLEWIGWIDPENGDTEYAPKFQGKATMTADTSPNTAYLQLSSLTSEDTAVYYCNGVYYGSRGFFDYWGQGTTLTVSS

SEQ ID NO: 206 - DNA, 360 bp, synthetic construct
  source 1..360: mol_type = other DNA
gaggttcagctgcagcagtctggggcagagcttgtgaggtcaggggcctcagtcaagttgtcctgcacagcttctggcttcaacattaaagactactatatgcactgggtgaagcagaggcctgatcagggcctggagtggattggatggattgatcctgagaatggtgatactgaatacgccccgaagttccagggcaaggccactatgactgcagacacatcccccaacacagcctacctgcagctcagcagcctgacatctgaggacactgccgtctattactgtaatggagtttactacggtagtagagggttctttgactactggggccaaggcaccactctcacagtctcctca

SEQ ID NO: 207 - protein, 112 aa, Mus musculus
DVVMTQTPLTLSVTIGQPASISCKSSQSLLDSDGKTYLNWLLQRPGQSPKRLIYLVSKLDSGVPDRFTGSGSGTDFTLKISRVEAEDLGVYYCCQITHFPFTFGSGTKLEIK

SEQ ID NO: 208 - DNA, 336 bp, synthetic construct
  source 1..336: mol_type = other DNA
gatgttgtgatgacccagactccactcactttgtcggttaccattggacaaccagcctccatctcttgcaagtcaagtcagagcctcttagatagtgatggaaagacatatttgaattggttgttacagaggccaggccagtctccaaagcgcctaatctatctggtgtctaaactggactctggagtccctgacaggttcactggcagtggatcagggacagatttcacactgaaaatcagcagagtggaggctgaggatttgggagtttattattgctgccaaattacacattttccattcacgttcggctcggggacaaagttggaaataaaa

SEQ ID NO: 209 - protein, 572 aa, Homo sapiens
MECLYYFLGFLLLAARLPLDAAKRFHDVLGNERPSAYMREHNQLNGWSSDENDWNEKLYPVWKRGDMRWKNSWKGGRVQAVLTSDSPALVGSNITFAVNLIFPRCQKEDANGNIVYEKNCRNEAGLSADPYVYNWTAWSEDSDGENGTGQSHHNVFPDGKPFPHHPGWRRWNFIYVFHTLGQYFQKLGRCSVRVSVNTANVTLGPQLMEVTVYRRHGRAYVPIAQVKDVYVVTDQIPVFVTMFQKNDRNSSDETFLKDLPIMFDVLIHDPSHFLNYSTINYKWSFGDNTGLFVSTNHTVNHTYVLNGTFSLNLTVKAAAPGPCPPPPPPPRPSKPTPSLATTLKSYDSNTPGPAGDNPLELSRIPDENCQINRYGHFQATITIVEGILEVNIIQMTDVLMPVPWPESSLIDFVVTCQGSIPTEVCTIISDPTCEITQNTVCSPVDVDEMCLLTVRRTFNGSGTYCVNLTLGDDTSLALTSTLISVPDRDPASPLRMANSALISVGCLAIFVTVISLLVYKKHKEYNPIENSPGNVVRSKGLSVFLNRAKAVFFPGNQEKDPLLKNQEFKGVS

SEQ ID NO: 210 - DNA, 1716 bp, Homo sapiens
  source 1..1716: mol_type = genomic DNA
atggaatgtctctactatttcctgggatttctgctcctggctgcaagattgccacttgatgccgccaaacgatttcatgatgtgctgggcaatgaaagaccttctgcttacatgagggagcacaatcaattaaatggctggtcttctgatgaaaatgactggaatgaaaaactctacccagtgtggaagcggggagacatgaggtggaaaaactcctggaagggaggccgtgtgcaggcggtcctgaccagtgactcaccagccctcgtgggctcaaatataacatttgcggtgaacctgatattccctagatgccaaaaggaagatgccaatggcaacatagtctatgagaagaactgcagaaatgaggctggtttatctgctgatccgtatgtttacaactggacagcatggtcagaggacagtgacggggaaaatggcaccggccaaagccatcataacgtcttccctgatgggaaaccttttcctcaccaccccggatggagaagatggaatttcatctacgtcttccacacacttggtcagtatttccagaaattgggacgatgttcagtgagagtttctgtgaacacagccaatgtgacacttgggcctcaactcatggaagtgactgtctacagaagacatggacgggcatatgttcccatcgcacaagtgaaagatgtgtacgtggtaacagatcagattcctgtgtttgtgactatgttccagaagaacgatcgaaattcatccgacgaaaccttcctcaaagatctccccattatgtttgatgtcctgattcatgatcctagccacttcctcaattattctaccattaactacaagtggagcttcggggataatactggcctgtttgtttccaccaatcatactgtgaatcacacgtatgtgctcaatggaaccttcagccttaacctcactgtgaaagctgcagcaccaggaccttgtccgccaccgccaccaccacccagaccttcaaaacccaccccttctttagcaactactctaaaatcttatgattcaaacaccccaggacctgctggtgacaaccccctggagctgagtaggattcctgatgaaaactgccagattaacagatatggccactttcaagccaccatcacaattgtagagggaatcttagaggttaacatcatccagatgacagacgtcctgatgccggtgccatggcctgaaagctccctaatagactttgtcgtgacctgccaagggagcattcccacggaggtctgtaccatcatttctgaccccacctgcgagatcacccagaacacagtctgcagccctgtggatgtggatgagatgtgtctgctgactgtgagacgaaccttcaatgggtctgggacgtactgtgtgaacctcaccctgggggatgacacaagcctggctctcacgagcaccctgatttctgttcctgacagagacccagcctcgcctttaaggatggcaaacagcgccctgatctccgttggctgcttggccatatttgtcactgtgatctccctcttggtgtacaaaaaacacaaggaatacaacccaatagaaaatagtcctgggaatgtggtcagaagcaaaggcctgagtgtctttctcaaccgtgcaaaagccgtgttcttcccgggaaaccaggaaaaggatccgctactcaaaaaccaagaatttaaaggagtttct

SEQ ID NO: 211 - protein, 574 aa, Mus musculus
MESLCGVLGFLLLAAGLPLQAAKRFRDVLGHEQYPNHMREHNQLRGWSSDENEWDEHLYPVWRRGDGRWKDSWEGGRVQAVLTSDSPALVGSNITFVVNLVFPRCQKEDANGNIVYEKNCRNDLGLTSDLHVYNWTAGADDGDWEDGTSRSQHLRFPDRRPFPRPHGWKKWSFVYVFHTLGQYFQKLGRCSARVSINTVNLTAGPQVMEVTVFRRYGRAYIPISKVKDVYVITDQIPVFVTMSQKNDRNLSDEIFLRDLPIVFDVLIHDPSHFLNDSAISYKWNFGDNTGLFVSNNHTLNHTYVLNGTFNLNLTVQTAVPGPCPPPSPSTPPPPSTPPSPPPSPLPTLSTPSPSLMPTGYKSMELSDISNENCRINRYGYFRATITIVEGILEVSIMQIADVPMPTPQPANSLMDFTVTCKGATPMEACTIISDPTCQIAQNRVCSPVAVDGLCLLSVRRAFNGSGTYCVNFTLGDDASLALTSTLISIPGKDPDSPLRAVNGVLISIGCLAVLVTMVTILLYKKHKAYKPIGNCPRNTVKGKGLSVLLSHAKAPFFRGDQEKDPLLQDKPRTL

SEQ ID NO: 212 - DNA, 1722 bp, Mus musculus
  source 1..1722: mol_type = genomic DNA
atggaaagtctctgcggggtcctgggatttctgctgctggctgcaggactgcctctccaggctgccaagcgatttcgtgatgtgctgggccatgaacagtatcccaatcacatgagagagcacaaccaattacgtggctggtcttcggatgaaaatgaatgggatgaacacctgtatccagtgtggaggaggggagacggcaggtggaaggactcctgggaaggaggccgtgtgcaggcagtcctgaccagtgactcaccggctctggtgggttccaatatcacctttgtggtgaacctggtgttccccagatgccagaaggaagatgctaatggcaatatcgtctatgagaagaactgcaggaatgatttgggactgacctctgacctgcatgtctacaactggactgcaggggcagatgatggtgactgggaagatggcaccagccgaagccagcatctcaggttcccggacaggaggcccttccctcgcccccatggatggaagaaatggagctttgtctacgtctttcacacacttggccagtatttccaaaaactgggtcggtgttcagcacgggtttctataaacacagtcaacttgacagctggccctcaggtcatggaagtgactgtctttcgaagatacggccgggcatacattcccatctcgaaggtgaaagatgtgtatgtgataacagatcagatccctgtattcgtgaccatgtcccagaagaatgacaggaacttgtctgatgagatcttcctcagagacctccccatcgtcttcgatgtcctcattcatgatcccagccacttcctcaacgactctgccatttcctacaagtggaactttggggacaacactggcctgtttgtctccaacaatcacactttgaatcacacttatgtgctcaatggaaccttcaaccttaacctcaccgtgcaaactgcagtgcccgggccatgccctcccccttcgccttcgactccgcctccaccttcaactccgccctcacctccgccctcacctctgcccacattatcaacacctagcccctctttaatgcctactggttacaaatccatggagctgagtgacatttccaatgaaaactgccgaataaacagatatggctacttcagagccaccatcacaattgtagaggggatcctggaagtcagcatcatgcagatagcagatgtccccatgcccacaccgcagcctgccaactccctgatggacttcactgtgacctgcaaaggggccacccccatggaagcctgtacgatcatctccgaccccacctgccagatcgcccagaaccgggtctgcagccctgtggctgtggatgggctgtgcctgctgtctgtgagaagagccttcaatgggtctggcacctactgtgtgaatttcactctgggagatgatgcaagcctggccctcaccagcaccctgatctctatccctggcaaagacccagactcccctctgagagcagtgaatggtgtcctgatctccattggctgcctggctgtgcttgtcaccatggttaccatcttgctgtacaaaaaacacaaggcgtacaagccaataggaaactgccccaggaacacggtcaagggcaaaggcctgagtgttctcctcagccacgcgaaagccccgttcttccgaggagaccaggagaaggatccattgctccaggacaagccaaggacactc

SEQ ID NO: 213 - protein, 572 aa, Rattus norvegicus
MESLCGVLVFLLLAAGLPLQAAKRFRDVLGHEQYPDHMRENNQLRGWSSDENEWDEQLYPVWRRGEGRWKDSWEGGRVQAALTSDSPALVGSNITFVVNLVFPRCQKEDANGNIVYERNCRSDLELASDPYVYNWTTGADDEDWEDSTSQGQHLRFPDGKPFPRPHGRKKWNFVYVFHTLGQYFQKLGRCSARVSINTVNLTVGPQVMEVIVFRRHGRAYIPISKVKDVYVITDQIPIFVTMYQKNDRNSSDETFLRDLPIFFDVLIHDPSHFLNYSAISYKWNFGDNTGLFVSNNHTLNHTYVLNGTFNFNLTVQTAVPGPCPSPTPSPSSSTSPSPASSPSPTLSTPSPSLMPTGHKSMELSDISNENCRINRYGYFRATITIVDGILEVNIIQVADVPIPTPQPDNSLMDFIVTCKGATPTEACTIISDPTCQIAQNRVCSPVAVDELCLLSVRRAFNGSGTYCVNFTLGDDASLALTSALISIPGKDLGSPLRTVNGVLISIGCLAMFVTMVTILLYKKHKTYKPIGNCTRNVVKGKGLSVFLSHAKAPFSRGDREKDPLLQDKPWML

SEQ ID NO: 214 - DNA, 1716 bp, Rattus norvegicus
  source 1..1716: mol_type = genomic DNA
atggaaagtctctgcggggtcctggtatttctgctgctggctgcaggactgccgctccaggcggccaagcggttccgtgatgtgctgggccatgagcagtatccggatcacatgagggagaacaaccaattacgtggctggtcttcagatgaaaatgaatgggatgaacagctgtatccagtgtggaggaggggagagggcagatggaaggactcctgggaaggaggccgtgtgcaggcagccctaaccagtgattcaccggccttggtgggttccaatatcaccttcgtagtgaacctggtgttccccagatgccagaaggaagatgccaacggcaatatcgtctatgagaggaactgcagaagtgatttggagctggcttctgacccgtatgtctacaactggaccacaggggcagacgatgaggactgggaagacagcaccagccaaggccagcacctcaggttccccgacgggaagcccttccctcgcccccacggacggaagaaatggaacttcgtctacgtcttccacacacttggtcagtattttcaaaagctgggtcggtgttcagcacgagtttctataaacacagtcaacttgacagttggccctcaggtcatggaagtgattgtctttcgaagacacggccgggcatacattcccatctccaaagtgaaagacgtgtatgtgataacagatcagatccctatattcgtgaccatgtaccagaagaatgaccggaactcgtctgatgaaaccttcctcagagacctccccattttcttcgatgtcctcattcacgatcccagtcatttcctcaactactctgccatttcctacaagtggaactttggggacaacactggcctgtttgtctccaacaatcacactttgaatcacacgtatgtgctcaatggaaccttcaactttaacctcaccgtgcaaactgcagtgccgggaccatgcccctcacccacaccttcgccttcttcttcgacttctccttcgcctgcatcttcgccttcacccacattatcaacacctagtccctctttaatgcctactggccacaaatccatggagctgagtgacatttccaatgaaaactgccgaataaacagatatggttacttcagagccaccatcacaattgtagatggaatcctagaagtcaacatcatccaggtagcagatgtcccaatccccacaccgcagcctgacaactcactgatggacttcattgtgacctgcaaaggggccactcccacggaagcctgtacgatcatctctgaccccacctgccagatcgcccagaacagggtgtgcagcccggtggctgtggatgagctgtgcctcctgtccgtgaggagagccttcaatgggtccggcacgtactgtgtgaatttcactctgggagacgatgcaagcctggccctcaccagcgccctgatctctatccctggcaaagacctaggctcccctctgagaacagtgaatggtgtcctgatctccattggctgcctggccatgtttgtcaccatggttaccatcttgctgtacaaaaaacacaagacgtacaagccaataggaaactgcaccaggaacgtggtcaagggcaaaggcctgagtgtttttctcagccatgcaaaagccccgttctcccgaggagaccgggagaaggatccactgctccaggacaagccatggatgctc

SEQ ID NO: 215 - protein, 498 aa, Homo sapiens
MECLYYFLGFLLLAARLPLDAAKRFHDVLGNERPSAYMREHNQLNGWSSDENDWNEKLYPVWKRGDMRWKNSWKGGRVQAVLTSDSPALVGSNITFAVNLIFPRCQKEDANGNIVYEKNCRNEAGLSADPYVYNWTAWSEDSDGENGTGQSHHNVFPDGKPFPHHPGWRRWNFIYVFHTLGQYFQKLGRCSVRVSVNTANVTLGPQLMEVTVYRRHGRAYVPIAQVKDVYVVTDQIPVFVTMFQKNDRNSSDETFLKDLPIMFDVLIHDPSHFLNYSTINYKWSFGDNTGLFVSTNHTVNHTYVLNGTFSLNLTVKAAAPGPCPPPPPPPRPSKPTPSLATTLKSYDSNTPGPAGDNPLELSRIPDENCQINRYGHFQATITIVEGILEVNIIQMTDVLMPVPWPESSLIDFVVTCQGSIPTEVCTIISDPTCEITQNTVCSPVDVDEMCLLTVRRTFNGSGTYCVNLTLGDDTSLALTSTLISVPDRDPASPLRMAN

SEQ ID NO: 216 - DNA, 1494 bp, Homo sapiens
  source 1..1494: mol_type = genomic DNA
atggaatgtctctactatttcctgggatttctgctcctggctgcaagattgccacttgatgccgccaaacgatttcatgatgtgctgggcaatgaaagaccttctgcttacatgagggagcacaatcaattaaatggctggtcttctgatgaaaatgactggaatgaaaaactctacccagtgtggaagcggggagacatgaggtggaaaaactcctggaagggaggccgtgtgcaggcggtcctgaccagtgactcaccagccctcgtgggctcaaatataacatttgcggtgaacctgatattccctagatgccaaaaggaagatgccaatggcaacatagtctatgagaagaactgcagaaatgaggctggtttatctgctgatccgtatgtttacaactggacagcatggtcagaggacagtgacggggaaaatggcaccggccaaagccatcataacgtcttccctgatgggaaaccttttcctcaccaccccggatggagaagatggaatttcatctacgtcttccacacacttggtcagtatttccagaaattgggacgatgttcagtgagagtttctgtgaacacagccaatgtgacacttgggcctcaactcatggaagtgactgtctacagaagacatggacgggcatatgttcccatcgcacaagtgaaagatgtgtacgtggtaacagatcagattcctgtgtttgtgactatgttccagaagaacgatcgaaattcatccgacgaaaccttcctcaaagatctccccattatgtttgatgtcctgattcatgatcctagccacttcctcaattattctaccattaactacaagtggagcttcggggataatactggcctgtttgtttccaccaatcatactgtgaatcacacgtatgtgctcaatggaaccttcagccttaacctcactgtgaaagctgcagcaccaggaccttgtccgccaccgccaccaccacccagaccttcaaaacccaccccttctttagcaactactctaaaatcttatgattcaaacaccccaggacctgctggtgacaaccccctggagctgagtaggattcctgatgaaaactgccagattaacagatatggccactttcaagccaccatcacaattgtagagggaatcttagaggttaacatcatccagatgacagacgtcctgatgccggtgccatggcctgaaagctccctaatagactttgtcgtgacctgccaagggagcattcccacggaggtctgtaccatcatttctgaccccacctgcgagatcacccagaacacagtctgcagccctgtggatgtggatgagatgtgtctgctgactgtgagacgaaccttcaatgggtctgggacgtactgtgtgaacctcaccctgggggatgacacaagcctggctctcacgagcaccctgatttctgttcctgacagagacccagcctcgcctttaaggatggcaaac

SEQ ID NO: 217 - protein, 502 aa, Mus musculus
MESLCGVLGFLLLAAGLPLQAAKRFRDVLGHEQYPDHMREHNQLRGWSSDENEWDEHLYPVWRRGDGRWKDSWEGGRVQAVLTSDSPALVGSNITFVVNLVFPRCQKEDANGNIVYEKNCRNDLGLTSDLHVYNWTAGADDGDWEDGTSRSQHLRFPDRRPFPRPHGWKKWSFVYVFHTLGQYFQKLGRCSARVSINTVNLTAGPQVMEVTVFRRYGRAYIPISKVKDVYVITDQIPVFVTMSQKNDRNLSDEIFLRDLPIVFDVLIHDPSHFLNDSAISYKWNFGDNTGLFVSNNHTLNHTYVLNGTFNLNLTVQTAVPGPCPPPSPSTPPPPSTPPSPPPSPLPTLSTPSPSLMPTGYKSMELSDISNENCRINRYGYFRATITIVEGILEVSIMQIADVPMPTPQPANSLMDFTVTCKGATPMEACTIISDPTCQIAQNRVCSPVAVDGLCLLSVRRAFNGSGTYCVNFTLGDDASLALTSTLISIPGKDPDSPLRAVN

SEQ ID NO: 218 - DNA, 1506 bp, Mus musculus
  source 1..1506: mol_type = genomic DNA
atggaaagtctctgcggggtcctgggatttctgctgctggctgcaggactgcctctccaggctgccaagcgatttcgtgatgtgctgggccatgaacagtatcccgatcacatgagagagcacaaccaattacgtggctggtcttcggatgaaaatgaatgggatgaacacctgtatccagtgtggaggaggggagacggcaggtggaaggactcctgggaaggaggccgtgtgcaggcagtcctgaccagtgactcaccggctctggtgggttccaatatcacttttgtggtgaacctggtgttccccagatgccagaaggaagatgctaatggcaatatcgtctatgagaagaactgcaggaatgatttgggactgacatctgacctgcatgtctacaactggactgcaggggcagatgatggtgactgggaagatggcaccagccgaagccagcatctcaggttcccggacaggaggcccttccctcgcccccatggatggaagaaatggagctttgtctacgtctttcacacacttggccagtatttccaaaaactgggtcggtgttcagcacgggtttctataaacacagtcaacttgacagctggccctcaggtcatggaagtgactgtctttcgaagatacggccgggcatacattcccatctcgaaggtgaaagatgtgtatgtgataacagatcagatccctgtattcgtgaccatgtcccagaagaatgacaggaacttgtctgatgagatcttcctcagagacctccccatcgtcttcgatgtcctcattcatgatcccagccacttcctcaacgactctgccatttcctacaagtggaactttggggacaacactggcctgtttgtctccaacaatcacactttgaatcacacttatgtgctcaatggaaccttcaaccttaacctcaccgtgcaaactgcagtgcccgggccatgccctcccccttcgccttcgactccgcctccaccttcaactccgccctcacctccgccctcacctctgcccacattatcaacacctagcccctctttaatgcctactggttacaaatccatggagctgagtgacatttccaatgaaaactgccgaataaacagatatggctacttcagagccaccatcacaattgtagaggggatcctggaagtcagcatcatgcagatagcagatgtccccatgcccacaccgcagcctgccaactccctgatggacttcactgtgacctgcaaaggggccacccccatggaagcctgtacgatcatctccgaccccacctgccagatcgcccagaaccgggtctgcagccctgtggctgtggatgggctgtgcctgctgtctgtgagaagagccttcaatgggtctggcacctactgtgtgaatttcactctgggagatgatgcaagcctggccctcaccagcaccctgatctctatccctggcaaagacccagactcccctctgagagcagtgaat

SEQ ID NO: 219 - protein, 500 aa, Rattus norvegicus
MESLCGVLVFLLLAAGLPLQAAKRFRDVLGHEQYPDHMRENNQLRGWSSDENEWDEQLYPVWRRGEGRWKDSWEGGRVQAALTSDSPALVGSNITFVVNLVFPRCQKEDANGNIVYERNCRSDLELASDPYVYNWTTGADDEDWEDNTSQGQHLRFPDGKPFPRPHGRKKWNFVYVFHTLGQYFQKLGQCSARVSINTVNLTVGPQVMEVIVFRRHGRAYIPISKVKDVYVITDQIPIFVTMYQKNDRNSSDETFLRDLPIFFDVLIHDPSHFLNYSAISYKWNFGDNTGLFVSNNHTLNHTYVLNGTFNFNLTVQTAVPGPCPSPTPSPSSSTSPSPASSPSPTLSTPSPSLMPTGYKSMELSDISNENCRINRYGYFRATITIVDGILEVNIIQVADVPIPTLQPDNSLMDFIVTCKGATPTEACTIISDPTCQIAQNRVCSPVAVDELCLLSVRRAFNGSGTYCVNFTLGDDASLALTSALISIPGKDLGSPLRTVN

SEQ ID NO: 220 - DNA, 1500 bp, Rattus norvegicus
  source 1..1500: mol_type = genomic DNA
atggaaagtctctgcggggtcctggtatttctgctgctggctgcaggactgccgctccaggcggccaagcggttccgtgatgtgctgggccatgagcagtatccggatcacatgagggagaacaaccaattacgtggctggtcttcagatgaaaatgaatgggatgaacagctgtatccagtgtggaggaggggagagggcagatggaaggactcctgggaaggaggccgtgtgcaggcagccctaaccagtgattcaccggccttggtgggttccaatatcaccttcgtagtgaacctggtgttccccagatgccagaaggaagatgccaacggcaatatcgtctatgagaggaactgcagaagtgatttggagctggcttctgacccgtatgtctacaactggaccacaggggcagacgatgaggactgggaagacaacaccagccaaggccagcacctcaggttccccgacgggaagcccttccctcgcccccacggacggaagaaatggaacttcgtctacgtcttccacacacttggtcagtattttcaaaagctgggtcagtgttcagcacgagtttctataaacacagtcaacttgacagttggccctcaggtcatggaagtgattgtctttcgaagacacggccgggcatacattcccatctccaaagtgaaagacgtgtatgtgataacagatcagatccctatattcgtgaccatgtaccagaagaatgaccggaactcgtctgatgaaaccttcctcagagacctccccattttcttcgatgtcctcattcacgatcccagtcatttcctcaactactctgccatttcctacaagtggaactttggggacaacactggcctgtttgtctccaacaatcacactttgaatcacacgtatgtgctcaatggaaccttcaactttaacctcaccgtgcaaactgcagtgccgggaccatgcccctcacccacaccttcgccttcttcttcgacttctccttcgcctgcatcttcgccttcacccacattatcaacacctagtccctctttaatgcctactggctacaaatccatggagctgagtgacatttccaatgaaaactgccgaataaacagatatggttacttcagagccaccatcacaattgtagatggaatcctagaagtcaacatcatccaggtagcagatgtcccaatccccacactgcagcctgacaactcactgatggacttcattgtgacctgcaaaggggccactcccacggaagcctgtacgatcatctctgaccccacctgccagatcgcccagaacagggtgtgcagcccggtggctgtggatgagctgtgcctcctgtccgtgaggagagccttcaatgggtccggcacgtactgtgtgaatttcactctgggagacgatgcaagcctggccctcaccagcgccctgatctctatccctggcaaagacctaggctcccctctgagaacagtgaat

SEQ ID NO: 221 - protein, 516 aa, synthetic construct
MECLYYFLGFLLLAARLPLDAAKRFHDVLGNERPSAYMREHNQLNGWSSDENDWNEKLYPVWKRGDMRWKNSWKGGRVQAVLTSDSPALVGSNITFAVNLIFPRCQKEDANGNIVYEKNCRNEAGLSADPYVYNWTAWSEDSDGENGTGQSHHNVFPDGKPFPHHPGWRRWNFIYVFHTLGQYFQKLGRCSVRVSVNTANVTLGPQLMEVTVYRRHGRAYVPIAQVKDVYVVTDQIPVFVTMFQKNDRNSSDETFLKDLPIMFDVLIHDPSHFLNYSTINYKWSFGDNTGLFVSTNHTVNHTYVLNGTFSLNLTVKAAAPGPCPPPPPPPRPSKPTPSLATTLKSYDSNTPGPAGDNPLELSRIPDENCQINRYGHFQATITIVEGILEVNIIQMTDVLMPVPWPESSLIDFVVTCQGSIPTEVCTIISDPTCEITQNTVCSPVDVDEMCLLTVRRTFNGSGTYCVNLTLGDDTSLALTSTLISVPDRDPASPLRMANEFDYKDDDDKLEHHHHHH

SEQ ID NO: 222 - DNA, 1548 bp, synthetic construct
  source 1..1548: mol_type = other DNA
atggaatgtctctactatttcctgggatttctgctcctggctgcaagattgccacttgatgccgccaaacgatttcatgatgtgctgggcaatgaaagaccttctgcttacatgagggagcacaatcaattaaatggctggtcttctgatgaaaatgactggaatgaaaaactctacccagtgtggaagcggggagacatgaggtggaaaaactcctggaagggaggccgtgtgcaggcggtcctgaccagtgactcaccagccctcgtgggctcaaatataacatttgcggtgaacctgatattccctagatgccaaaaggaagatgccaatggcaacatagtctatgagaagaactgcagaaatgaggctggtttatctgctgatccgtatgtttacaactggacagcatggtcagaggacagtgacggggaaaatggcaccggccaaagccatcataacgtcttccctgatgggaaaccttttcctcaccaccccggatggagaagatggaatttcatctacgtcttccacacacttggtcagtatttccagaaattgggacgatgttcagtgagagtttctgtgaacacagccaatgtgacacttgggcctcaactcatggaagtgactgtctacagaagacatggacgggcatatgttcccatcgcacaagtgaaagatgtgtacgtggtaacagatcagattcctgtgtttgtgactatgttccagaagaacgatcgaaattcatccgacgaaaccttcctcaaagatctccccattatgtttgatgtcctgattcatgatcctagccacttcctcaattattctaccattaactacaagtggagcttcggggataatactggcctgtttgtttccaccaatcatactgtgaatcacacgtatgtgctcaatggaaccttcagccttaacctcactgtgaaagctgcagcaccaggaccttgtccgccaccgccaccaccacccagaccttcaaaacccaccccttctttagcaactactctaaaatcttatgattcaaacaccccaggacctgctggtgacaaccccctggagctgagtaggattcctgatgaaaactgccagattaacagatatggccactttcaagccaccatcacaattgtagagggaatcttagaggttaacatcatccagatgacagacgtcctgatgccggtgccatggcctgaaagctccctaatagactttgtcgtgacctgccaagggagcattcccacggaggtctgtaccatcatttctgaccccacctgcgagatcacccagaacacagtctgcagccctgtggatgtggatgagatgtgtctgctgactgtgagacgaaccttcaatgggtctgggacgtactgtgtgaacctcaccctgggggatgacacaagcctggctctcacgagcaccctgatttctgttcctgacagagacccagcctcgcctttaaggatggcaaacgaattcgattataaggatgacgatgacaagctcgagcatcaccaccatcaccac

SEQ ID NO: 223 - protein, 520 aa, synthetic construct
MESLCGVLGFLLLAAGLPLQAAKRFRDVLGHEQYPDHMREHNQLRGWSSDENEWDEHLYPVWRRGDGRWKDSWEGGRVQAVLTSDSPALVGSNITFVVNLVFPRCQKEDANGNIVYEKNCRNDLGLTSDLHVYNWTAGADDGDWEDGTSRSQHLRFPDRRPFPRPHGWKKWSFVYVFHTLGQYFQKLGRCSARVSINTVNLTAGPQVMEVTVFRRYGRAYIPISKVKDVYVITDQIPVFVTMSQKNDRNLSDEIFLRDLPIVFDVLIHDPSHFLNDSAISYKWNFGDNTGLFVSNNHTLNHTYVLNGTFNLNLTVQTAVPGPCPPPSPSTPPPPSTPPSPPPSPLPTLSTPSPSLMPTGYKSMELSDISNENCRINRYGYFRATITIVEGILEVSIMQIADVPMPTPQPANSLMDFTVTCKGATPMEACTIISDPTCQIAQNRVCSPVAVDGLCLLSVRRAFNGSGTYCVNFTLGDDASLALTSTLISIPGKDPDSPLRAVNEFDYKDDDDKLEHHHHHH

SEQ ID NO: 224 - DNA, 1560 bp, synthetic construct
  source 1..1560: mol_type = other DNA
atggaaagtctctgcggggtcctgggatttctgctgctggctgcaggactgcctctccaggctgccaagcgatttcgtgatgtgctgggccatgaacagtatcccgatcacatgagagagcacaaccaattacgtggctggtcttcggatgaaaatgaatgggatgaacacctgtatccagtgtggaggaggggagacggcaggtggaaggactcctgggaaggaggccgtgtgcaggcagtcctgaccagtgactcaccggctctggtgggttccaatatcacttttgtggtgaacctggtgttccccagatgccagaaggaagatgctaatggcaatatcgtctatgagaagaactgcaggaatgatttgggactgacatctgacctgcatgtctacaactggactgcaggggcagatgatggtgactgggaagatggcaccagccgaagccagcatctcaggttcccggacaggaggcccttccctcgcccccatggatggaagaaatggagctttgtctacgtctttcacacacttggccagtatttccaaaaactgggtcggtgttcagcacgggtttctataaacacagtcaacttgacagctggccctcaggtcatggaagtgactgtctttcgaagatacggccgggcatacattcccatctcgaaggtgaaagatgtgtatgtgataacagatcagatccctgtattcgtgaccatgtcccagaagaatgacaggaacttgtctgatgagatcttcctcagagacctccccatcgtcttcgatgtcctcattcatgatcccagccacttcctcaacgactctgccatttcctacaagtggaactttggggacaacactggcctgtttgtctccaacaatcacactttgaatcacacttatgtgctcaatggaaccttcaaccttaacctcaccgtgcaaactgcagtgcccgggccatgccctcccccttcgccttcgactccgcctccaccttcaactccgccctcacctccgccctcacctctgcccacattatcaacacctagcccctctttaatgcctactggttacaaatccatggagctgagtgacatttccaatgaaaactgccgaataaacagatatggctacttcagagccaccatcacaattgtagaggggatcctggaagtcagcatcatgcagatagcagatgtccccatgcccacaccgcagcctgccaactccctgatggacttcactgtgacctgcaaaggggccacccccatggaagcctgtacgatcatctccgaccccacctgccagatcgcccagaaccgggtctgcagccctgtggctgtggatgggctgtgcctgctgtctgtgagaagagccttcaatgggtctggcacctactgtgtgaatttcactctgggagatgatgcaagcctggccctcaccagcaccctgatctctatccctggcaaagacccagactcccctctgagagcagtgaatgaattcgattataaggatgacgatgacaagctcgagcatcaccaccatcaccac

SEQ ID NO: 225 - protein, 518 aa, synthetic construct
MESLCGVLVFLLLAAGLPLQAAKRFRDVLGHEQYPDHMRENNQLRGWSSDENEWDEQLYPVWRRGEGRWKDSWEGGRVQAALTSDSPALVGSNITFVVNLVFPRCQKEDANGNIVYERNCRSDLELASDPYVYNWTTGADDEDWEDNTSQGQHLRFPDGKPFPRPHGRKKWNFVYVFHTLGQYFQKLGQCSARVSINTVNLTVGPQVMEVIVFRRHGRAYIPISKVKDVYVITDQIPIFVTMYQKNDRNSSDETFLRDLPIFFDVLIHDPSHFLNYSAISYKWNFGDNTGLFVSNNHTLNHTYVLNGTFNFNLTVQTAVPGPCPSPTPSPSSSTSPSPASSPSPTLSTPSPSLMPTGYKSMELSDISNENCRINRYGYFRATITIVDGILEVNIIQVADVPIPTLQPDNSLMDFIVTCKGATPTEACTIISDPTCQIAQNRVCSPVAVDELCLLSVRRAFNGSGTYCVNFTLGDDASLALTSALISIPGKDLGSPLRTVNEFDYKDDDDKLEHHHHHH

SEQ ID NO: 226 - DNA, 1554 bp, synthetic construct
  source 1..1554: mol_type = other DNA
atggaaagtctctgcggggtcctggtatttctgctgctggctgcaggactgccgctccaggcggccaagcggttccgtgatgtgctgggccatgagcagtatccggatcacatgagggagaacaaccaattacgtggctggtcttcagatgaaaatgaatgggatgaacagctgtatccagtgtggaggaggggagagggcagatggaaggactcctgggaaggaggccgtgtgcaggcagccctaaccagtgattcaccggccttggtgggttccaatatcaccttcgtagtgaacctggtgttccccagatgccagaaggaagatgccaacggcaatatcgtctatgagaggaactgcagaagtgatttggagctggcttctgacccgtatgtctacaactggaccacaggggcagacgatgaggactgggaagacaacaccagccaaggccagcacctcaggttccccgacgggaagcccttccctcgcccccacggacggaagaaatggaacttcgtctacgtcttccacacacttggtcagtattttcaaaagctgggtcagtgttcagcacgagtttctataaacacagtcaacttgacagttggccctcaggtcatggaagtgattgtctttcgaagacacggccgggcatacattcccatctccaaagtgaaagacgtgtatgtgataacagatcagatccctatattcgtgaccatgtaccagaagaatgaccggaactcgtctgatgaaaccttcctcagagacctccccattttcttcgatgtcctcattcacgatcccagtcatttcctcaactactctgccatttcctacaagtggaactttggggacaacactggcctgtttgtctccaacaatcacactttgaatcacacgtatgtgctcaatggaaccttcaactttaacctcaccgtgcaaactgcagtgccgggaccatgcccctcacccacaccttcgccttcttcttcgacttctccttcgcctgcatcttcgccttcacccacattatcaacacctagtccctctttaatgcctactggctacaaatccatggagctgagtgacatttccaatgaaaactgccgaataaacagatatggttacttcagagccaccatcacaattgtagatggaatcctagaagtcaacatcatccaggtagcagatgtcccaatccccacactgcagcctgacaactcactgatggacttcattgtgacctgcaaaggggccactcccacggaagcctgtacgatcatctctgaccccacctgccagatcgcccagaacagggtgtgcagcccggtggctgtggatgagctgtgcctcctgtccgtgaggagagccttcaatgggtccggcacgtactgtgtgaatttcactctgggagacgatgcaagcctggccctcaccagcgccctgatctctatccctggcaaagacctaggctcccctctgagaacagtgaatgaattcgattataaggatgacgatgacaagctcgagcatcaccaccatcaccac

SEQ ID NO: 227 - protein, 269 aa, synthetic construct
MECLYYFLGFLLLAARLPLDAAKRFHDVLGNERPSAYMREHNQLNGWSSDENDWNEKLYPVWKRGDMRWKNSWKGGRVQAVLTSDSPALVGSNITFAVNLIFPRCQKEDANGNIVYEKNCRNEAGLSADPYVYNWTAWSEDSDGENGTGQSHHNVFPDGKPFPHHPGWRRWNFIYVFHTLGQYFQKLGRCSVRVSVNTANVTLGPQLMEVTVYRRHGRAYVPIAQVKDVYVVTDQIPVFVTMFQKNDRNSSEFDYKDDDDKLEHHHHHH

SEQ ID NO: 228 - DNA, 807 bp, synthetic construct
  source 1..807: mol_type = other DNA
atggaatgtctctactatttcctgggatttctgctcctggctgcaagattgccacttgatgccgccaaacgatttcatgatgtgctgggcaatgaaagaccttctgcttacatgagggagcacaatcaattaaatggctggtcttctgatgaaaatgactggaatgaaaaactctacccagtgtggaagcggggagacatgaggtggaaaaactcctggaagggaggccgtgtgcaggcggtcctgaccagtgactcaccagccctcgtgggctcaaatataacatttgcggtgaacctgatattccctagatgccaaaaggaagatgccaatggcaacatagtctatgagaagaactgcagaaatgaggctggtttatctgctgatccgtatgtttacaactggacagcatggtcagaggacagtgacggggaaaatggcaccggccaaagccatcataacgtcttccctgatgggaaaccttttcctcaccaccccggatggagaagatggaatttcatctacgtcttccacacacttggtcagtatttccagaaattgggacgatgttcagtgagagtttctgtgaacacagccaatgtgacacttgggcctcaactcatggaagtgactgtctacagaagacatggacgggcatatgttcccatcgcacaagtgaaagatgtgtacgtggtaacagatcagattcctgtgtttgtgactatgttccagaagaacgatcgaaattcatccgaattcgattataaggatgacgatgacaagctcgagcatcaccaccatcaccac

SEQ ID NO: 229 - protein, 339 aa, synthetic construct
MECLYYFLGFLLLAARLPLDAAKRFHDVLGNERPSAYMREHNQLNGWSSDENDWNEKLYPVWKRGDMRWKNSWKGGRVQAVLTSDSPALVGSNITFAVNLIFPRCQKEDANGNIVYEKNCRNEAGLSADPYVYNWTAWSEDSDGENGTGQSHHNVFPDGKPFPHHPGWRRWNFIYVFHTLGQYFQKLGRCSVRVSVNTANVTLGPQLMEVTVYRRHGRAYVPIAQVKDVYVVTDQIPVFVTMFQKNDRNSSDETFLKDLPIMFDVLIHDPSHFLNYSTINYKWSFGDNTGLFVSTNHTVNHTYVLNGTFSLNLTVKAAAPGEFDYKDDDDKLEHHHHHH

SEQ ID NO: 230 - DNA, 1017 bp, synthetic construct
  source 1..1017: mol_type = other DNA
atggaatgtctctactatttcctgggatttctgctcctggctgcaagattgccacttgatgccgccaaacgatttcatgatgtgctgggcaatgaaagaccttctgcttacatgagggagcacaatcaattaaatggctggtcttctgatgaaaatgactggaatgaaaaactctacccagtgtggaagcggggagacatgaggtggaaaaactcctggaagggaggccgtgtgcaggcggtcctgaccagtgactcaccagccctcgtgggctcaaatataacatttgcggtgaacctgatattccctagatgccaaaaggaagatgccaatggcaacatagtctatgagaagaactgcagaaatgaggctggtttatctgctgatccgtatgtttacaactggacagcatggtcagaggacagtgacggggaaaatggcaccggccaaagccatcataacgtcttccctgatgggaaaccttttcctcaccaccccggatggagaagatggaatttcatctacgtcttccacacacttggtcagtatttccagaaattgggacgatgttcagtgagagtttctgtgaacacagccaatgtgacacttgggcctcaactcatggaagtgactgtctacagaagacatggacgggcatatgttcccatcgcacaagtgaaagatgtgtacgtggtaacagatcagattcctgtgtttgtgactatgttccagaagaacgatcgaaattcatccgacgaaaccttcctcaaagatctccccattatgtttgatgtcctgattcatgatcctagccacttcctcaattattctaccattaactacaagtggagcttcggggataatactggcctgtttgtttccaccaatcatactgtgaatcacacgtatgtgctcaatggaaccttcagccttaacctcactgtgaaagctgcagcaccaggagaattcgattataaggatgacgatgacaagctcgagcatcaccaccatcaccac

SEQ ID NO: 231 - protein, 393 aa, synthetic construct
MECLYYFLGFLLLAARLPLDAAKRFHDVLGNERPSAYMREHNQLNGWSSDENDWNEKLYPVWKRGDMRWKNSWKGGRVQAVLTSDSPALVGSNITFAVNLIFPRCQKEDANGNIVYEKNCRNEAGLSADPYVYNWTAWSEDSDGENGTGQSHHNVFPDGKPFPHHPGWRRWNFIYVFHTLGQYFQKLGRCSVRVSVNTANVTLGPQLMEVTVYRRHGRAYVPIAQVKDVYVVTDQIPVFVTMFQKNDRNSSDETFLKDLPIMFDVLIHDPSHFLNYSTINYKWSFGDNTGLFVSTNHTVNHTYVLNGTFSLNLTVKAAAPGPCPPPPPPPRPSKPTPSLATTLKSYDSNTPGPAGDNPLELSRIPDENCQINRYGEFDYKDDDDKLEHHHHHH

SEQ ID NO: 232 - DNA, 1179 bp, synthetic construct
  source 1..1179: mol_type = other DNA
atggaatgtctctactatttcctgggatttctgctcctggctgcaagattgccacttgatgccgccaaacgatttcatgatgtgctgggcaatgaaagaccttctgcttacatgagggagcacaatcaattaaatggctggtcttctgatgaaaatgactggaatgaaaaactctacccagtgtggaagcggggagacatgaggtggaaaaactcctggaagggaggccgtgtgcaggcggtcctgaccagtgactcaccagccctcgtgggctcaaatataacatttgcggtgaacctgatattccctagatgccaaaaggaagatgccaatggcaacatagtctatgagaagaactgcagaaatgaggctggtttatctgctgatccgtatgtttacaactggacagcatggtcagaggacagtgacggggaaaatggcaccggccaaagccatcataacgtcttccctgatgggaaaccttttcctcaccaccccggatggagaagatggaatttcatctacgtcttccacacacttggtcagtatttccagaaattgggacgatgttcagtgagagtttctgtgaacacagccaatgtgacacttgggcctcaactcatggaagtgactgtctacagaagacatggacgggcatatgttcccatcgcacaagtgaaagatgtgtacgtggtaacagatcagattcctgtgtttgtgactatgttccagaagaacgatcgaaattcatccgacgaaaccttcctcaaagatctccccattatgtttgatgtcctgattcatgatcctagccacttcctcaattattctaccattaactacaagtggagcttcggggataatactggcctgtttgtttccaccaatcatactgtgaatcacacgtatgtgctcaatggaaccttcagccttaacctcactgtgaaagctgcagcaccaggaccttgtccgccaccgccaccaccacccagaccttcaaaacccaccccttctttagcaactactctaaaatcttatgattcaaacaccccaggacctgctggtgacaaccccctggagctgagtaggattcctgatgaaaactgccagattaacagatatggcgaattcgattataaggatgacgatgacaagctcgagcatcaccaccatcaccac

SEQ ID NO: 233 - protein, 436 aa, synthetic construct
MECLYYFLGFLLLAARLPLDAAKRFHDVLGNERPSAYMREHNQLNGWSSDENDWNEKLYPVWKRGDMRWKNSWKGGRVQAVLTSDSPALVGSNITFAVNLIFPRCQKEDANGNIVYEKNCRNEAGLSADPYVYNWTAWSEDSDGENGTGQSHHNVFPDGKPFPHHPGWRRWNFIYVFHTLGQYFQKLGRCSVRVSVNTANVTLGPQLMEVTVYRRHGRAYVPIAQVKDVYVVTDQIPVFVTMFQKNDRNSSDETFLKDLPIMFDVLIHDPSHFLNYSTINYKWSFGDNTGLFVSTNHTVNHTYVLNGTFSLNLTVKAAAPGPCPPPPPPPRPSKPTPSLATTLKSYDSNTPGPAGDNPLELSRIPDENCQINRYGHFQATITIVEGILEVNIIQMTDVLMPVPWPESSLIDFVVTCQGEFDYKDDDDKLEHHHHHH

SEQ ID NO: 234 - DNA, 1308 bp, synthetic construct
  source 1..1308: mol_type = other DNA
atggaatgtctctactatttcctgggatttctgctcctggctgcaagattgccacttgatgccgccaaacgatttcatgatgtgctgggcaatgaaagaccttctgcttacatgagggagcacaatcaattaaatggctggtcttctgatgaaaatgactggaatgaaaaactctacccagtgtggaagcggggagacatgaggtggaaaaactcctggaagggaggccgtgtgcaggcggtcctgaccagtgactcaccagccctcgtgggctcaaatataacatttgcggtgaacctgatattccctagatgccaaaaggaagatgccaatggcaacatagtctatgagaagaactgcagaaatgaggctggtttatctgctgatccgtatgtttacaactggacagcatggtcagaggacagtgacggggaaaatggcaccggccaaagccatcataacgtcttccctgatgggaaaccttttcctcaccaccccggatggagaagatggaatttcatctacgtcttccacacacttggtcagtatttccagaaattgggacgatgttcagtgagagtttctgtgaacacagccaatgtgacacttgggcctcaactcatggaagtgactgtctacagaagacatggacgggcatatgttcccatcgcacaagtgaaagatgtgtacgtggtaacagatcagattcctgtgtttgtgactatgttccagaagaacgatcgaaattcatccgacgaaaccttcctcaaagatctccccattatgtttgatgtcctgattcatgatcctagccacttcctcaattattctaccattaactacaagtggagcttcggggataatactggcctgtttgtttccaccaatcatactgtgaatcacacgtatgtgctcaatggaaccttcagccttaacctcactgtgaaagctgcagcaccaggaccttgtccgccaccgccaccaccacccagaccttcaaaacccaccccttctttagcaactactctaaaatcttatgattcaaacaccccaggacctgctggtgacaaccccctggagctgagtaggattcctgatgaaaactgccagattaacagatatggccactttcaagccaccatcacaattgtagagggaatcttagaggttaacatcatccagatgacagacgtcctgatgccggtgccatggcctgaaagctccctaatagactttgtcgtgacctgccaaggggaattcgattataaggatgacgatgacaagctcgagcatcaccaccatcaccac

SEQ ID NO: 235 - protein, 465 aa, synthetic construct
MECLYYFLGFLLLAARLPLDAAGSGRVQAVLTSDSPALVGSNITFAVNLIFPRCQKEDANGNIVYEKNCRNEAGLSADPYVYNWTAWSEDSDGENGTGQSHHNVFPDGKPFPHHPGWRRWNFIYVFHTLGQYFQKLGRCSVRVSVNTANVTLGPQLMEVTVYRRHGRAYVPIAQVKDVYVVTDQIPVFVTMFQKNDRNSSDETFLKDLPIMFDVLIHDPSHFLNYSTINYKWSFGDNTGLFVSTNHTVNHTYVLNGTFSLNLTVKAAAPGPCPPPPPPPRPSKPTPSLATTLKSYDSNTPGPAGDNPLELSRIPDENCQINRYGHFQATITIVEGILEVNIIQMTDVLMPVPWPESSLIDFVVTCQGSIPTEVCTIISDPTCEITQNTVCSPVDVDEMCLLTVRRTFNGSGTYCVNLTLGDDTSLALTSTLISVPDRDPASPLRMANEFDYKDDDDKLEHHHHHH

SEQ ID NO: 236 - DNA, 1395 bp, synthetic construct
  source 1..1395: mol_type = other DNA
atggaatgtctctactatttcctgggatttctgctcctggctgcaagattgccacttgatgccgccggatccggccgtgtgcaggcggtcctgaccagtgactcaccagccctcgtgggctcaaatataacatttgcggtgaacctgatattccctagatgccaaaaggaagatgccaatggcaacatagtctatgagaagaactgcagaaatgaggctggtttatctgctgatccgtatgtttacaactggacagcatggtcagaggacagtgacggggaaaatggcaccggccaaagccatcataacgtcttccctgatgggaaaccttttcctcaccaccccggatggagaagatggaatttcatctacgtcttccacacacttggtcagtatttccagaaattgggacgatgttcagtgagagtttctgtgaacacagccaatgtgacacttgggcctcaactcatggaagtgactgtctacagaagacatggacgggcatatgttcccatcgcacaagtgaaagatgtgtacgtggtaacagatcagattcctgtgtttgtgactatgttccagaagaacgatcgaaattcatccgacgaaaccttcctcaaagatctccccattatgtttgatgtcctgattcatgatcctagccacttcctcaattattctaccattaactacaagtggagcttcggggataatactggcctgtttgtttccaccaatcatactgtgaatcacacgtatgtgctcaatggaaccttcagccttaacctcactgtgaaagctgcagcaccaggaccttgtccgccaccgccaccaccacccagaccttcaaaacccaccccttctttagcaactactctaaaatcttatgattcaaacaccccaggacctgctggtgacaaccccctggagctgagtaggattcctgatgaaaactgccagattaacagatatggccactttcaagccaccatcacaattgtagagggaatcttagaggttaacatcatccagatgacagacgtcctgatgccggtgccatggcctgaaagctccctaatagactttgtcgtgacctgccaagggagcattcccacggaggtctgtaccatcatttctgaccccacctgcgagatcacccagaacacagtctgcagccctgtggatgtggatgagatgtgtctgctgactgtgagacgaaccttcaatgggtctgggacatactgtgtgaacctcaccctgggggatgacacaagcctggctctcacgagcaccctgatttctgttcctgacagagacccagcctcgcctttaaggatggcaaacgaattcgattataaggatgacgatgacaagctcgagcatcaccaccatcaccac

SEQ ID NO: 237 - protein, 430 aa, synthetic construct
MECLYYFLGFLLLAARLPLDAAKRFHDVLGNERPSAYMREHNQLNGWSSDENDWNEKLYPVWKRGDMRWKNSWKGGRVQAVLTSDSPALVGSNITFAVNLIFPRCQKEDANGNIVYEKNCRNEAGLSADPYVYNWTAWSEDSDGENGTGQSHHNVFPDGKPFPHHPGWRRWNFIYVFHTLGQYFQKLGRCSVRVSVNTANVTLGPQLMEVTVYRRHGRAYVPIAQVKDVYVVTDQIPVFVTMFQKNDRNSSDETFLKDLPIMFDVLIHDPSHFLNYSTINYKWSFGDNTGLFVSTNHTVNHTYVLNGTFSLNLTVKAAAPGPCPPPPPPPRPSKPTPSLATTLKSYDSNTPGPAGDNPLELSRIPDENCQINRYGHFQATITIVEGILEVNIIQMTDVLMPVPWPESSLIDFEFDYKDDDDKLEHHHHHH

SEQ ID NO: 238 - DNA, 1290 bp, synthetic construct
  source 1..1290: mol_type = other DNA
atggaatgtctctactatttcctgggatttctgctcctggctgcaagattgccacttgatgccgccaaacgatttcatgatgtgctgggcaatgaaagaccttctgcttacatgagggagcacaatcaattaaatggctggtcttctgatgaaaatgactggaatgaaaaactctacccagtgtggaagcggggagacatgaggtggaaaaactcctggaagggaggccgtgtgcaggcggtcctgaccagtgactcaccagccctcgtgggctcaaatataacatttgcggtgaacctgatattccctagatgccaaaaggaagatgccaatggcaacatagtctatgagaagaactgcagaaatgaggctggtttatctgctgatccgtatgtttacaactggacagcatggtcagaggacagtgacggggaaaatggcaccggccaaagccatcataacgtcttccctgatgggaaaccttttcctcaccaccccggatggagaagatggaatttcatctacgtcttccacacacttggtcagtatttccagaaattgggacgatgttcagtgagagtttctgtgaacacagccaatgtgacacttgggcctcaactcatggaagtgactgtctacagaagacatggacgggcatatgttcccatcgcacaagtgaaagatgtgtacgtggtaacagatcagattcctgtgtttgtgactatgttccagaagaacgatcgaaattcatccgacgaaaccttcctcaaagatctccccattatgtttgatgtcctgattcatgatcctagccacttcctcaattattctaccattaactacaagtggagcttcggggataatactggcctgtttgtttccaccaatcatactgtgaatcacacgtatgtgctcaatggaaccttcagccttaacctcactgtgaaagctgcagcaccaggaccttgtccgccaccgccaccaccacccagaccttcaaaacccaccccttctttagcaactactctaaaatcttatgattcaaacaccccaggacctgctggtgacaaccccctggagctgagtaggattcctgatgaaaactgccagattaacagatatggccactttcaagccaccatcacaattgtagagggaatcttagaggttaacatcatccagatgacagacgtcctgatgccggtgccatggcctgaaagctccctaatagactttgaattcgattataaggatgacgatgacaagctcgagcatcaccaccatcaccac

SEQ ID NO: 239 - protein, 424 aa, synthetic construct
MECLYYFLGFLLLAARLPLDAAKRFHDVLGNERPSAYMREHNQLNGWSSDENDWNEKLYPVWKRGDMRWKNSWKGGRVQAVLTSDSPALVGSNITFAVNLIFPRCQKEDANGNIVYEKNCRNEAGLSADPYVYNWTAWSEDSDGENGTGQSHHNVFPDGKPFPHHPGWRRWNFIYVFHTLGQYFQKLGRCSVRVSVNTANVTLGPQLMEVTVYRRHGRAYVPIAQVKDVYVVTDQIPVFVTMFQKNDRNSSDETFLKDLPIMFDVLIHDPSHFLNYSTINYKWSFGDNTGLFVSTNHTVNHTYVLNGTFSLNLTVKAAAPGPCPPPPPPPRPSKPTPSLATTLKSYDSNTPGPAGDNPLELSRIPDENCQINRYGHFQATITIVEGILEVNIIQMTDVLMPVPWPEEFDYKDDDDKLEHHHHHH

SEQ ID NO: 240 - DNA, 1272 bp, synthetic construct
  source 1..1272: mol_type = other DNA
atggaatgtctctactatttcctgggatttctgctcctggctgcaagattgccacttgatgccgccaaacgatttcatgatgtgctgggcaatgaaagaccttctgcttacatgagggagcacaatcaattaaatggctggtcttctgatgaaaatgactggaatgaaaaactctacccagtgtggaagcggggagacatgaggtggaaaaactcctggaagggaggccgtgtgcaggcggtcctgaccagtgactcaccagccctcgtgggctcaaatataacatttgcggtgaacctgatattccctagatgccaaaaggaagatgccaatggcaacatagtctatgagaagaactgcagaaatgaggctggtttatctgctgatccgtatgtttacaactggacagcatggtcagaggacagtgacggggaaaatggcaccggccaaagccatcataacgtcttccctgatgggaaaccttttcctcaccaccccggatggagaagatggaatttcatctacgtcttccacacacttggtcagtatttccagaaattgggacgatgttcagtgagagtttctgtgaacacagccaatgtgacacttgggcctcaactcatggaagtgactgtctacagaagacatggacgggcatatgttcccatcgcacaagtgaaagatgtgtacgtggtaacagatcagattcctgtgtttgtgactatgttccagaagaacgatcgaaattcatccgacgaaaccttcctcaaagatctccccattatgtttgatgtcctgattcatgatcctagccacttcctcaattattctaccattaactacaagtggagcttcggggataatactggcctgtttgtttccaccaatcatactgtgaatcacacgtatgtgctcaatggaaccttcagccttaacctcactgtgaaagctgcagcaccaggaccttgtccgccaccgccaccaccacccagaccttcaaaacccaccccttctttagcaactactctaaaatcttatgattcaaacaccccaggacctgctggtgacaaccccctggagctgagtaggattcctgatgaaaactgccagattaacagatatggccactttcaagccaccatcacaattgtagagggaatcttagaggttaacatcatccagatgacagacgtcctgatgccggtgccatggcctgaagaattcgattataaggatgacgatgacaagctcgagcatcaccaccatcaccac

SEQ ID NO: 241 - protein, 418 aa, synthetic construct
MECLYYFLGFLLLAARLPLDAAKRFHDVLGNERPSAYMREHNQLNGWSSDENDWNEKLYPVWKRGDMRWKNSWKGGRVQAVLTSDSPALVGSNITFAVNLIFPRCQKEDANGNIVYEKNCRNEAGLSADPYVYNWTAWSEDSDGENGTGQSHHNVFPDGKPFPHHPGWRRWNFIYVFHTLGQYFQKLGRCSVRVSVNTANVTLGPQLMEVTVYRRHGRAYVPIAQVKDVYVVTDQIPVFVTMFQKNDRNSSDETFLKDLPIMFDVLIHDPSHFLNYSTINYKWSFGDNTGLFVSTNHTVNHTYVLNGTFSLNLTVKAAAPGPCPPPPPPPRPSKPTPSLATTLKSYDSNTPGPAGDNPLELSRIPDENCQINRYGHFQATITIVEGILEVNIIQMTDVLMEFDYKDDDDKLEHHHHHH

SEQ ID NO: 242 - DNA, 1254 bp, synthetic construct
  source 1..1254: mol_type = other DNA
atggaatgtctctactatttcctgggatttctgctcctggctgcaagattgccacttgatgccgccaaacgatttcatgatgtgctgggcaatgaaagaccttctgcttacatgagggagcacaatcaattaaatggctggtcttctgatgaaaatgactggaatgaaaaactctacccagtgtggaagcggggagacatgaggtggaaaaactcctggaagggaggccgtgtgcaggcggtcctgaccagtgactcaccagccctcgtgggctcaaatataacatttgcggtgaacctgatattccctagatgccaaaaggaagatgccaatggcaacatagtctatgagaagaactgcagaaatgaggctggtttatctgctgatccgtatgtttacaactggacagcatggtcagaggacagtgacggggaaaatggcaccggccaaagccatcataacgtcttccctgatgggaaaccttttcctcaccaccccggatggagaagatggaatttcatctacgtcttccacacacttggtcagtatttccagaaattgggacgatgttcagtgagagtttctgtgaacacagccaatgtgacacttgggcctcaactcatggaagtgactgtctacagaagacatggacgggcatatgttcccatcgcacaagtgaaagatgtgtacgtggtaacagatcagattcctgtgtttgtgactatgttccagaagaacgatcgaaattcatccgacgaaaccttcctcaaagatctccccattatgtttgatgtcctgattcatgatcctagccacttcctcaattattctaccattaactacaagtggagcttcggggataatactggcctgtttgtttccaccaatcatactgtgaatcacacgtatgtgctcaatggaaccttcagccttaacctcactgtgaaagctgcagcaccaggaccttgtccgccaccgccaccaccacccagaccttcaaaacccaccccttctttagcaactactctaaaatcttatgattcaaacaccccaggacctgctggtgacaaccccctggagctgagtaggattcctgatgaaaactgccagattaacagatatggccactttcaagccaccatcacaattgtagagggaatcttagaggttaacatcatccagatgacagacgtcctgatggaattcgattataaggatgacgatgacaagctcgagcatcaccaccatcaccac

SEQ ID NO: 243 - protein, 412 aa, synthetic construct
MECLYYFLGFLLLAARLPLDAAKRFHDVLGNERPSAYMREHNQLNGWSSDENDWNEKLYPVWKRGDMRWKNSWKGGRVQAVLTSDSPALVGSNITFAVNLIFPRCQKEDANGNIVYEKNCRNEAGLSADPYVYNWTAWSEDSDGENGTGQSHHNVFPDGKPFPHHPGWRRWNFIYVFHTLGQYFQKLGRCSVRVSVNTANVTLGPQLMEVTVYRRHGRAYVPIAQVKDVYVVTDQIPVFVTMFQKNDRNSSDETFLKDLPIMFDVLIHDPSHFLNYSTINYKWSFGDNTGLFVSTNHTVNHTYVLNGTFSLNLTVKAAAPGPCPPPPPPPRPSKPTPSLATTLKSYDSNTPGPAGDNPLELSRIPDENCQINRYGHFQATITIVEGILEVNIIQEFDYKDDDDKLEHHHHHH

SEQ ID NO: 244 - DNA, 1236 bp, synthetic construct
  source 1..1236: mol_type = other DNA
atggaatgtctctactatttcctgggatttctgctcctggctgcaagattgccacttgatgccgccaaacgatttcatgatgtgctgggcaatgaaagaccttctgcttacatgagggagcacaatcaattaaatggctggtcttctgatgaaaatgactggaatgaaaaactctacccagtgtggaagcggggagacatgaggtggaaaaactcctggaagggaggccgtgtgcaggcggtcctgaccagtgactcaccagccctcgtgggctcaaatataacatttgcggtgaacctgatattccctagatgccaaaaggaagatgccaatggcaacatagtctatgagaagaactgcagaaatgaggctggtttatctgctgatccgtatgtttacaactggacagcatggtcagaggacagtgacggggaaaatggcaccggccaaagccatcataacgtcttccctgatgggaaaccttttcctcaccaccccggatggagaagatggaatttcatctacgtcttccacacacttggtcagtatttccagaaattgggacgatgttcagtgagagtttctgtgaacacagccaatgtgacacttgggcctcaactcatggaagtgactgtctacagaagacatggacgggcatatgttcccatcgcacaagtgaaagatgtgtacgtggtaacagatcagattcctgtgtttgtgactatgttccagaagaacgatcgaaattcatccgacgaaaccttcctcaaagatctccccattatgtttgatgtcctgattcatgatcctagccacttcctcaattattctaccattaactacaagtggagcttcggggataatactggcctgtttgtttccaccaatcatactgtgaatcacacgtatgtgctcaatggaaccttcagccttaacctcactgtgaaagctgcagcaccaggaccttgtccgccaccgccaccaccacccagaccttcaaaacccaccccttctttagcaactactctaaaatcttatgattcaaacaccccaggacctgctggtgacaaccccctggagctgagtaggattcctgatgaaaactgccagattaacagatatggccactttcaagccaccatcacaattgtagagggaatcttagaggttaacatcatccaggaattcgattataaggatgacgatgacaagctcgagcatcaccaccatcaccac

SEQ ID NO: 245 - protein, 406 aa, synthetic construct
MECLYYFLGFLLLAARLPLDAAKRFHDVLGNERPSAYMREHNQLNGWSSDENDWNEKLYPVWKRGDMRWKNSWKGGRVQAVLTSDSPALVGSNITFAVNLIFPRCQKEDANGNIVYEKNCRNEAGLSADPYVYNWTAWSEDSDGENGTGQSHHNVFPDGKPFPHHPGWRRWNFIYVFHTLGQYFQKLGRCSVRVSVNTANVTLGPQLMEVTVYRRHGRAYVPIAQVKDVYVVTDQIPVFVTMFQKNDRNSSDETFLKDLPIMFDVLIHDPSHFLNYSTINYKWSFGDNTGLFVSTNHTVNHTYVLNGTFSLNLTVKAAAPGPCPPPPPPPRPSKPTPSLATTLKSYDSNTPGPAGDNPLELSRIPDENCQINRYGHFQATITIVEGILEFDYKDDDDKLEHHHHHH

SEQ ID NO: 246 - DNA, 1218 bp, synthetic construct
  source 1..1218: mol_type = other DNA
atggaatgtctctactatttcctgggatttctgctcctggctgcaagattgccacttgatgccgccaaacgatttcatgatgtgctgggcaatgaaagaccttctgcttacatgagggagcacaatcaattaaatggctggtcttctgatgaaaatgactggaatgaaaaactctacccagtgtggaagcggggagacatgaggtggaaaaactcctggaagggaggccgtgtgcaggcggtcctgaccagtgactcaccagccctcgtgggctcaaatataacatttgcggtgaacctgatattccctagatgccaaaaggaagatgccaatggcaacatagtctatgagaagaactgcagaaatgaggctggtttatctgctgatccgtatgtttacaactggacagcatggtcagaggacagtgacggggaaaatggcaccggccaaagccatcataacgtcttccctgatgggaaaccttttcctcaccaccccggatggagaagatggaatttcatctacgtcttccacacacttggtcagtatttccagaaattgggacgatgttcagtgagagtttctgtgaacacagccaatgtgacacttgggcctcaactcatggaagtgactgtctacagaagacatggacgggcatatgttcccatcgcacaagtgaaagatgtgtacgtggtaacagatcagattcctgtgtttgtgactatgttccagaagaacgatcgaaattcatccgacgaaaccttcctcaaagatctccccattatgtttgatgtcctgattcatgatcctagccacttcctcaattattctaccattaactacaagtggagcttcggggataatactggcctgtttgtttccaccaatcatactgtgaatcacacgtatgtgctcaatggaaccttcagccttaacctcactgtgaaagctgcagcaccaggaccttgtccgccaccgccaccaccacccagaccttcaaaacccaccccttctttagcaactactctaaaatcttatgattcaaacaccccaggacctgctggtgacaaccccctggagctgagtaggattcctgatgaaaactgccagattaacagatatggccactttcaagccaccatcacaattgtagagggaatcttagaattcgattataaggatgacgatgacaagctcgagcatcaccaccatcaccac

SEQ ID NO: 247 - protein, 400 aa, synthetic construct
MECLYYFLGFLLLAARLPLDAAKRFHDVLGNERPSAYMREHNQLNGWSSDENDWNEKLYPVWKRGDMRWKNSWKGGRVQAVLTSDSPALVGSNITFAVNLIFPRCQKEDANGNIVYEKNCRNEAGLSADPYVYNWTAWSEDSDGENGTGQSHHNVFPDGKPFPHHPGWRRWNFIYVFHTLGQYFQKLGRCSVRVSVNTANVTLGPQLMEVTVYRRHGRAYVPIAQVKDVYVVTDQIPVFVTMFQKNDRNSSDETFLKDLPIMFDVLIHDPSHFLNYSTINYKWSFGDNTGLFVSTNHTVNHTYVLNGTFSLNLTVKAAAPGPCPPPPPPPRPSKPTPSLATTLKSYDSNTPGPAGDNPLELSRIPDENCQINRYGHFQATITEFDYKDDDDKLEHHHHHH

SEQ ID NO: 248 - DNA, 1200 bp, synthetic construct
  source 1..1200: mol_type = other DNA
atggaatgtctctactatttcctgggatttctgctcctggctgcaagattgccacttgatgccgccaaacgatttcatgatgtgctgggcaatgaaagaccttctgcttacatgagggagcacaatcaattaaatggctggtcttctgatgaaaatgactggaatgaaaaactctacccagtgtggaagcggggagacatgaggtggaaaaactcctggaagggaggccgtgtgcaggcggtcctgaccagtgactcaccagccctcgtgggctcaaatataacatttgcggtgaacctgatattccctagatgccaaaaggaagatgccaatggcaacatagtctatgagaagaactgcagaaatgaggctggtttatctgctgatccgtatgtttacaactggacagcatggtcagaggacagtgacggggaaaatggcaccggccaaagccatcataacgtcttccctgatgggaaaccttttcctcaccaccccggatggagaagatggaatttcatctacgtcttccacacacttggtcagtatttccagaaattgggacgatgttcagtgagagtttctgtgaacacagccaatgtgacacttgggcctcaactcatggaagtgactgtctacagaagacatggacgggcatatgttcccatcgcacaagtgaaagatgtgtacgtggtaacagatcagattcctgtgtttgtgactatgttccagaagaacgatcgaaattcatccgacgaaaccttcctcaaagatctccccattatgtttgatgtcctgattcatgatcctagccacttcctcaattattctaccattaactacaagtggagcttcggggataatactggcctgtttgtttccaccaatcatactgtgaatcacacgtatgtgctcaatggaaccttcagccttaacctcactgtgaaagctgcagcaccaggaccttgtccgccaccgccaccaccacccagaccttcaaaacccaccccttctttagcaactactctaaaatcttatgattcaaacaccccaggacctgctggtgacaaccccctggagctgagtaggattcctgatgaaaactgccagattaacagatatggccactttcaagccaccatcacagaattcgattataaggatgacgatgacaagctcgagcatcaccaccatcaccac

SEQ ID NO: 249 - protein, 252 aa, synthetic construct
MECLYYFLGFLLLAARLPLDAAKRFHDVLGNERPSAYMREHNQLNGWSSDENDWNEKLYPVWKRGDMRWKNSWKGGRVQAVLTSDSPALVGSNITFAVNLIFPRCQKEDANGNIVYEKNCRNEAGLSADPYVYNWTAWSEDSDGENGTGQSHHNVFPDGKPFPHHPGWRRWNFIYVFHTLGQYFQKLGRCSVRVSVNTANVTLGPQLMEVTVYRRHGRAYVPIAQVKDVYVVTDEFDYKDDDDKLEHHHHHH

SEQ ID NO: 250 - DNA, 756 bp, synthetic construct
  source 1..756: mol_type = other DNA
atggaatgtctctactatttcctgggatttctgctcctggctgcaagattgccacttgatgccgccaaacgatttcatgatgtgctgggcaatgaaagaccttctgcttacatgagggagcacaatcaattaaatggctggtcttctgatgaaaatgactggaatgaaaaactctacccagtgtggaagcggggagacatgaggtggaaaaactcctggaagggaggccgtgtgcaggcggtcctgaccagtgactcaccagccctcgtgggctcaaatataacatttgcggtgaacctgatattccctagatgccaaaaggaagatgccaatggcaacatagtctatgagaagaactgcagaaatgaggctggtttatctgctgatccgtatgtttacaactggacagcatggtcagaggacagtgacggggaaaatggcaccggccaaagccatcataacgtcttccctgatgggaaaccttttcctcaccaccccggatggagaagatggaatttcatctacgtcttccacacacttggtcagtatttccagaaattgggacgatgttcagtgagagtttctgtgaacacagccaatgtgacacttgggcctcaactcatggaagtgactgtctacagaagacatggacgggcatatgttcccatcgcacaagtgaaagatgtgtacgtggtaacagatgaattcgattataaggatgacgatgacaagctcgagcatcaccaccatcaccac

SEQ ID NO: 251 - protein, 122 aa, synthetic construct; identical to SEQ ID NO: 29

SEQ ID NO: 252 - DNA, 366 bp, synthetic construct
  source 1..366: mol_type = other DNA
caggtccagctgcagcagcctggggccgaaatcgtgagacctggcgctagcgtgaagctgtcttgcaaggccagcggctacaccttcacagacaactggatgggctgggtgaagcagagacctggccagggcctggagtggatcggcgccatcgatccctccgacagcttcaccaattacaatcagaactttaagggcaaggccaccctgacagtggatacctcttccagcacagcttacatgcagctgtctagcctgacaagcgaggattctgccgtgtatttttgtacaagaagcggctattacggcagccctaagctgggcggcgactactggggccagggcaccacactgacagtgtcttcc

SEQ ID NO: 253 - protein, 106 aa, synthetic construct; identical to SEQ ID NO: 31

SEQ ID NO: 254 - DNA, 318 bp, synthetic construct
  source 1..318: mol_type = other DNA
cagattgtgctgactcagtcacccgctatcatgtccgcttctctgggcgaggagatcacactgacctgttctgcctccagctctatctcctacatgcactggtatcagcagaagtctggcacctctccaaagctgctgatctactccacctctaacctggcttctggcgtgccttccagattctctggcagcggctctggcaccttctattccctgacaatctccagcgtggaggctgaggatgccgctgactactattgccaccagtggaactcttacccatgcacatttggcggcggcacaaagctggagatcaag

SEQ ID NO: 255 - protein, 8 aa, Mus musculus
GLSLTSIN

SEQ ID NO: 256 - DNA, 24 bp, synthetic construct
  source 1..24: mol_type = other DNA
ggcctttccctgacgagcatcaac

SEQ ID NO: 257 - protein, 7 aa, Mus musculus
IWSDGDT

SEQ ID NO: 258 - DNA, 21 bp, synthetic construct
  source 1..21: mol_type = other DNA
atttggagtgatggggatact

SEQ ID NO: 259 - protein, 6 aa, Mus musculus
ARGIRD

SEQ ID NO: 260 - DNA, 18 bp, synthetic construct
  source 1..18: mol_type = other DNA
gctagaggcataagggac

SEQ ID NO: 261 - protein, 11 aa, Mus musculus
QSLKYSDGKTY

SEQ ID NO: 262 - DNA, 33 bp, synthetic construct
  source 1..33: mol_type = other DNA
cagtccctgaagtatagcgatgggaaaacctac

SEQ ID NO: 263-264 - skipped (2 entries)

SEQ ID NO: 265 - protein, 9 aa, Mus musculus
CQGSYSPHT

SEQ ID NO: 266 - DNA, 27 bp, synthetic construct
  source 1..27: mol_type = other DNA
tgtcaagggtcctattcaccccatacc

SEQ ID NO: 267 - protein, 112 aa, Mus musculus
QVQLKASGPGLVQPSQTLSLTCTVSGLSLTSININWIRQPPGKGLEWMGVIWSDGDTDFNSAVKSRLSISRDTSKSQVFLNMNSLQTEDTAMYFCARGIRDWGQGVMVTVSS

SEQ ID NO: 268 - DNA, 336 bp, synthetic construct
  source 1..336: mol_type = other DNA
caggtccagctgaaagccagtggtcctggactggttcagccaagccagaccctctcactcacatgcaccgtttctggcctttccctgacgagcatcaacatcaattggattcggcaaccacctggcaaaggattggagtggatgggcgtgatttggagtgatggggatactgacttcaactccgctgtgaagtcccgactgtccatttcacgcgataccagcaagtctcaggtgttcctgaacatgaatagcctgcagactgaggacactgccatgtacttctgtgctagaggcataagggactggggtcaaggagtcatggttaccgtgtcatct

SEQ ID NO: 269 - protein, 112 aa, Mus musculus
DIVMTQTPLSLSVAIGQSASISCKSSQSLKYSDGKTYLNWVFQSPGQSPKRLIYQVSKLDSGVPDRFSGTGSETDFTLKISRVEAEDLGVYYCCQGSYSPHTFGSGTKLEIK

SEQ ID NO: 270 - DNA, 336 bp, synthetic construct
  source 1..336: mol_type = other DNA
gacatagtgatgacccagacacccttgagtctgagtgttgccattggccaaagtgcctctatctcctgcaagtcaagtcagtccctgaagtatagcgatgggaaaacctacctgaactgggtctttcagagcccaggtcagtcacccaaacggctgatttaccaggtcagcaaactcgactctggagtaccagaccgcttttccggaacaggtagcgagactgacttcaccctcaagatctctagggtggaagccgaggatcttggcgtgtattactgctgtcaagggtcctattcaccccatacctttggttccggcacaaagctggagatcaag

SEQ ID NO: 271 - protein, 10 aa, synthetic construct
GYTFTDNWMG

SEQ ID NO: 272 - DNA, 30 bp, synthetic construct
  source 1..30: mol_type = other DNA
ggctacaccttcaccgataattggatgggc

SEQ ID NO: 273 - protein, 17 aa, synthetic construct
AIDPSDSFTNYNQNFKG

SEQ ID NO: 274 - DNA, 51 bp, synthetic construct
  source 1..51: mol_type = other DNA
gccatcgacccttctgactcctttaccaactacaaccagaacttcaagggc

SEQ ID NO: 275 - protein, 15 aa, synthetic construct
TRSGYYGSPKLGGDY

SEQ ID NO: 276 - DNA, 45 bp, synthetic construct
  source 1..45: mol_type = other DNA
accagatctggatactacggctctcccaagctgggaggcgactac

SEQ ID NO: 277 - protein, 10 aa, synthetic construct
SASSSISYMH

SEQ ID NO: 278 - DNA, 30 bp, synthetic construct
  source 1..30: mol_type = other DNA
tccgcctcctcctcaatctcctacatgcac

SEQ ID NO: 279 - protein, 7 aa, synthetic construct
STSNLAS

SEQ ID NO: 280 - DNA, 21 bp, synthetic construct
  source 1..21: mol_type = other DNA
tccacctccaacctggcctct

SEQ ID NO: 281 - protein, 9 aa, synthetic construct
HQWNSYPCT

SEQ ID NO: 282 - DNA, 27 bp, synthetic construct
  source 1..27: mol_type = other DNA
caccagtggaattcttacccctgcacc

SEQ ID NO: 283 - protein, 8 aa, synthetic construct
GYTFTDNW

SEQ ID NO: 284 - DNA, 24 bp, synthetic construct
  source 1..24: mol_type = other DNA
ggctacaccttcaccgataattgg

SEQ ID NO: 285 - protein, 8 aa, synthetic construct
IDPSDSFT

SEQ ID NO: 286 - DNA, 24 bp, synthetic construct
  source 1..24: mol_type = other DNA
atcgacccttctgactcctttacc

SEQ ID NO: 287 - protein, 15 aa, synthetic construct
TRSGYYGSPKLGGDY

SEQ ID NO: 288 - DNA, 45 bp, synthetic construct; identical to SEQ ID NO: 276
  source 1..45: mol_type = other DNA

SEQ ID NO: 289 - protein, 5 aa, synthetic construct
SSISY

SEQ ID NO: 290 - DNA, 15 bp, synthetic construct
  source 1..15: mol_type = other DNA
tcctcaatctcctac

SEQ ID NO: 291-292 - skipped (2 entries)

SEQ ID NO: 293 - protein, 9 aa, synthetic construct
HQWNSYPCT

SEQ ID NO: 294 - DNA, 27 bp, synthetic construct
  source 1..27: mol_type = other DNA
caccagtggaattcttacccctgcacc

SEQ ID NO: 295 - protein, 122 aa, synthetic construct
QVQLVQSGAEVKKPGASVKVSCKASGYTFTDNWMGWVKQRPGQGLEWIGAIDPSDSFTNYNQNFKGRVTMTVDTSISTAYMELSRLRSDDSAVYFCTRSGYYGSPKLGGDYWGQGTLVTVSS

SEQ ID NO: 296 - DNA, 366 bp, synthetic construct
  source 1..366: mol_type = other DNA
caggtgcagctggtccagtccggcgccgaggtgaagaagcccggcgctagcgtgaaagtgtcctgcaaggcctctggctacaccttcaccgataattggatgggctgggtcaagcagagacctggccaaggcctggaatggatcggcgccatcgacccttctgactcctttaccaactacaaccagaacttcaagggccgggtgaccatgacagtggatacctccatcagcaccgcctacatggaactgtccagactgagatccgacgacagcgctgtgtacttctgcaccagatctggatactacggctctcccaagctgggaggcgactactggggccagggcaccctggtgaccgtgtcctcc

SEQ ID NO: 297 - protein, 106 aa, synthetic construct
EIVLTQSPSSLSASVGDRVTITCSASSSISYMHWYQQKSGTAPKLLIYSTSNLASGVPSRFSGSGSGTDFTFTISSLQPEDAATYYCHQWNSYPCTFGGGTKLEIK

SEQ ID NO: 298 - DNA, 318 bp, synthetic construct
  source 1..318: mol_type = other DNA
gagatcgtgctgacccaatctccttcttctctgtctgcttccgtgggcgacagagtgaccatcacctgctccgcctcctcctcaatctcctacatgcactggtaccagcagaagtctggaacagctcctaaacttctgatctactccacctccaacctggcctctggcgtgccatctcgcttctccggctctggcagcggaaccgactttacatttaccatctctagcctgcagcctgaggacgccgctacatactactgccaccagtggaattcttacccctgcaccttcggcggcggcaccaagctggaaatcaag

SEQ ID NO: 299 - protein, 12 aa, synthetic construct
GFSLSTSVMGVG

SEQ ID NO: 300 - DNA, 36 bp, synthetic construct
  source 1..36: mol_type = other DNA
ggcttcagcctgtctacctccgtgatgggcgtgggc

SEQ ID NO: 301 - protein, 16 aa, synthetic construct
DIWWDDDKDYNPSLKS

SEQ ID NO: 302 - DNA, 48 bp, synthetic construct
  source 1..48: mol_type = other DNA
gacatctggtgggacgacgacaaggactacaatccctctctgaagtcc

SEQ ID NO: 303 - protein, 15 aa, synthetic construct
ARTYYSNYEYYGMDY

SEQ ID NO: 304 - DNA, 45 bp, synthetic construct
  source 1..45: mol_type = other DNA
gccagaacctactactccaactacgagtactacggcatggattac

SEQ ID NO: 305 - protein, 16 aa, synthetic construct
RSSQTIILSNGNTYLE

SEQ ID NO: 306 - DNA, 48 bp, synthetic construct
  source 1..48: mol_type = other DNA
agatcctctcagaccatcatcctgtccaacggcaacacctacctggaa

SEQ ID NO: 307 - protein, 7 aa, synthetic construct
KVSNRFS

SEQ ID NO: 308 - DNA, 21 bp, synthetic construct
  source 1..21: mol_type = other DNA
aaggtgtccaatcggttctct

SEQ ID NO: 309 - protein, 9 aa, synthetic construct
FQGSHVPFT

SEQ ID NO: 310 - DNA, 27 bp, synthetic construct
  source 1..27: mol_type = other DNA
ttccaaggctctcacgtgccctttacc

SEQ ID NO: 311 - protein, 10 aa, synthetic construct
GFSLSTSVMG

SEQ ID NO: 312 - DNA, 30 bp, synthetic construct
  source 1..30: mol_type = other DNA
ggcttcagcctgtctacctccgtgatgggc

SEQ ID NO: 313 - protein, 7 aa, synthetic construct
IWWDDDK

SEQ ID NO: 314 - DNA, 21 bp, synthetic construct
  source 1..21: mol_type = other DNA
atctggtgggacgacgacaag

SEQ ID NO: 315 - protein, 15 aa, synthetic construct
ARTYYSNYEYYGMDY

SEQ ID NO: 316 - DNA, 45 bp, synthetic construct; identical to SEQ ID NO: 304
  source 1..45: mol_type = other DNA

SEQ ID NO: 317 - protein, 11 aa, synthetic construct
QTIILSNGNTY

SEQ ID NO: 318 - DNA, 33 bp, synthetic construct
  source 1..33: mol_type = other DNA
cagaccatcatcctgagcaacggcaacacctac

SEQ ID NO: 319-320 - skipped (2 entries)

SEQ ID NO: 321 - protein, 9 aa, synthetic construct
FQGSHVPFT

SEQ ID NO: 322 - DNA, 27 bp, synthetic construct
  source 1..27: mol_type = other DNA
ttccagggctctcacgtgcccttcacc

SEQ ID NO: 323 - protein, 123 aa, synthetic construct
QVQLVQSGPGLVQPTQTLTLTCSFSGFSLSTSVMGVGWIRQPSGKGLEWLADIWWDDDKDYNPSLKSRLTISKDTSKNQVVLTMTNMDTVDTATYYCARTYYSNYEYYGMDYWGQGTLVTVSS

SEQ ID NO: 324 - DNA, 369 bp, synthetic construct
  source 1..369: mol_type = other DNA
caagtgcaactagtgcaaagtggtccaggtctggtgcagcctacccagaccctgacactgacctgtagcttctccggcttcagcctgtctacctccgtgatgggcgtgggctggatccggcaaccttctggcaagggcctggaatggctggccgacatctggtgggacgacgacaaggactacaatccctctctgaagtccagactgaccatctccaaagatacctctaagaaccaggtcgtgctgaccatgaccaacatggataccgtggacaccgctacatattactgcgccagaacctactactccaactacgagtactacggcatggattactggggccagggaacactcgtgaccgtgtcctct

SEQ ID NO: 325 - protein, 113 aa, synthetic construct
DIVMTQSPDSLAVSLGERATINCRSSQTIILSNGNTYLEWYQQKPGQPPKLLIYKVSNRFSGVPDRFSGSGSGTDFTLTISSLQAEDVAVYYCFQGSHVPFTFGSGTKLEIKR

SEQ ID NO: 326 - DNA, 339 bp, synthetic construct
  source 1..339: mol_type = other DNA
gatattgtgatgactcaaagtccagatagtctggctgtctctctgggcgagagagctacaatcaactgtagatcctctcagaccatcatcctgtccaacggcaacacctacctggaatggtatcagcagaaaccaggccagcctcctaagctgctgatctacaaggtgtccaatcggttctctggcgtgcctgatagattctccggctctggaagcggaaccgacttcaccctgaccatctccagcctgcaggccgaggacgtggccgtgtactactgcttccaaggctctcacgtgccctttaccttcggctccggcaccaagctggagatcaagcgg

SEQ ID NO: 327 - protein, 10 aa, synthetic construct
GYTFTTYWMN

SEQ ID NO: 328 - protein, 17 aa, synthetic construct
AINPSNDYTEYNQKFKD

SEQ ID NO: 329 - protein, 6 aa, synthetic construct
SYSPDY

SEQ ID NO: 330 - protein, 10 aa, synthetic construct
GYTFTTYWMN

SEQ ID NO: 331 - protein, 8 aa, synthetic construct
INPSNDYT

SEQ ID NO: 332 - protein, 8 aa, synthetic construct
GRSYSPDY

SEQ ID NO: 333 - protein, 115 aa, synthetic construct
QVQLVQSGAEVKKPGASVKVSCKASGYTFTTYWMNWVRQAPGQGLEWIGAINPSNDYTEYNQKFKDRVTMTADTSTSTVYMELSSLRSEDTAVYYCGRSYSPDYWGQGTTVTVSS

SEQ ID NO: 334 - protein, 10 aa, synthetic construct
GYTFTTYWMN

SEQ ID NO: 335 - protein, 17 aa, synthetic construct
AINPSNDYTEYNQKFKD

SEQ ID NO: 336 - protein, 6 aa, synthetic construct
SYSPDY

SEQ ID NO: 337 - protein, 10 aa, synthetic construct
GYTFTTYWMN

SEQ ID NO: 338 - protein, 8 aa, synthetic construct
INPSNDYT

SEQ ID NO: 339 - protein, 8 aa, synthetic construct
GRSYSPDY

SEQ ID NO: 340 - protein, 115 aa, synthetic construct
QVQLVQSGAEVKKPGASVKVSCKASGYTFTTYWMNWVRQAPGQGLEWIGAINPSNDYTEYNQKFKDRATMTADTSTSTVYMELSSLRSEDTAVYYCGRSYSPDYWGQGTTVTVSS

SEQ ID NO: 341 - protein, 10 aa, synthetic construct
GYTFTTYWMN

SEQ ID NO: 342 - protein, 17 aa, synthetic construct
AINPSNDYTEYNQKFKD

SEQ ID NO: 343 - protein, 6 aa, synthetic construct
SYSPDY

SEQ ID NO: 344 - protein, 10 aa, synthetic construct
GYTFTTYWMN

SEQ ID NO: 345 - protein, 8 aa, synthetic construct
INPSNDYT

SEQ ID NO: 346 - protein, 8 aa, synthetic construct
GRSYSPDY

SEQ ID NO: 347 - protein, 115 aa, synthetic construct
QVQLVQSGAEVKKPGASVKVSCKASGYTFTTYWMNWVRQAPGQGLEWIGAINPSNDYTEYNQKFKDRAIMTADKSTSTVYMELSSLRSEDTAVYYCGRSYSPDYWGQGTTVTVSS

SEQ ID NO: 348 - protein, 11 aa, synthetic construct
KASQNVDNHVA

SEQ ID NO: 349 - protein, 7 aa, synthetic construct
SASYRYS

SEQ ID NO: 350 - protein, 9 aa, synthetic construct
QQYKSYPFT

SEQ ID NO: 351 - protein, 6 aa, synthetic construct
QNVDNH

SEQ ID NO: 352 - skipped

SEQ ID NO: 353 - protein, 9 aa, synthetic construct
QQYKSYPFT

SEQ ID NO: 354 - protein, 107 aa, synthetic construct
DIQMTQSPSSLSASVGDRVTITCKASQNVDNHVAWFQQKPGKAPKALIYSASYRYSGVPSRFSGSGSGTDFTLTISSLQPEDFATYFCQQYKSYPFTFGGGTKLEIK

SEQ ID NO: 355 - protein, 11 aa, synthetic construct
KASQNVDNHVA

SEQ ID NO: 356 - protein, 7 aa, synthetic construct
SASYRYS

SEQ ID NO: 357 - protein, 9 aa, synthetic construct
QQYKSYPFT

SEQ ID NO: 358 - protein, 6 aa, synthetic construct
QNVDNH

SEQ ID NO: 359 - skipped

SEQ ID NO: 360 - protein, 9 aa, synthetic construct
QQYKSYPFT

SEQ ID NO: 361 - protein, 107 aa, synthetic construct
DIQMTQSPSSLSASVGDRVTITCKASQNVDNHVAWFQQKPGKAPKALIYSASYRYSGVPDRFSGSGSGTDFTLTISSLQPEDFATYFCQQYKSYPFTFGGGTKLEIK

SEQ ID NO: 362 - protein, 11 aa, synthetic construct
KASQNVDNHVA

SEQ ID NO: 363 - protein, 7 aa, synthetic construct
SASYRYS

SEQ ID NO: 364 - protein, 9 aa, synthetic construct
QQYKSYPFT

SEQ ID NO: 365 - protein, 6 aa, synthetic construct
QNVDNH

SEQ ID NO: 366 - skipped

SEQ ID NO: 367 - protein, 9 aa, synthetic construct
QQYKSYPFT

SEQ ID NO: 368 - protein, 107 aa, synthetic construct
DIQMTQSPSSLSASVGDRVTITCKASQNVDNHVAWHQQKPGKAPKALIYSASYRYSGVPDRFTGSGSGTDFTLTISSLQPEDFADYFCQQYKSYPFTFGGGTKLEIK